European Patent Application EP 4 484 557 A1, published January 1, 2025. Title: 카르바모일 인산 합성효소 라지 서브유닛 변이체 및 이를 이용한 L-오르니틴 생산 방법. Applicant: CJ CheilJedang Corporation. The sequence listing filed with the application follows.

SEQUENCE LISTING (57 sequences)

SEQ ID NO: 1 - protein, 1113 aa, unidentified
  REGION 1..1113: note = CarB
MPKRSDINHVLVIGSGPIVIGQACEFDYSGTQACRVLKEEGLRVTLINSNPATIMTDPEMADHTYVEPIEPEYIDKIFAKEIEQGHPIDAVLATLGGQTALNAAIQLDRLGILEKYGVELIGADIDAIERGEDRQKFKDIVTTIGGESARSRVCHNMDEVHETVAELGLPVVVRPSFTMGGLGSGLAYNTEDLERIAGGGLAASPEANVLIEESILGWKEFELELMRDTADNVVVICSIENVDALGVHTGDSVTVAPALTLTDREFQKMRDQGIAIIREVGVDTGGCNIQFAINPVDGRIITIEMNPRVSRSSALASKATGFPIAKMAAKLAIGYTLDEITNDITGETPAAFEPTIDYVVVKAPRFAFEKFVGADDTLTTTMKSVGEVMSLGRNYIAALNKALRSLETKQQGFWTKPDEFFAGERATDKAAVLEDLKRPTEGRLYDVELAMRLGASVEELYEASSIDPWFLAELEALVQFRQKLVDAPFLNEDLLREAKFMGLSDLQIAALRPEFAGEDGVRTLRLSLGIRPVFKTVDTCAAEFEAKTPYHYSAYELDPAAESEVAPQTEREKVLILGSGPNRIGQGIEFDYSCVHAALELSRVGYETVMVNCNPETVSTDYDTADRLYFEPLTFEDVMEVYHAEAQSGTVAGVIVQLGGQTPLGLADRLKKAGVPVIGTSPEAIDMAEDRGEFGALLNREQLPAPAFGTATSFEEARTVADEISYPVLVRPSYVLGGRGMEIVYDEASLEDYINRATELSSDHPVLVDRFLDNAIEIDVDALCDGDEVYLAGVMEHIEEAGIHSGDSACALPPMTLGAQDIEKVREATKKLALGIGVQGLMNVQYALKDDILYVIEANPRASRTVPFVSKATGVNLAKAASRIAVGATIKDLQDEGMIPTEYDGGSLPLDAPIAVKEAVLPFNRFRRPDGKTLDTLLSPEMKSTGEVMGLANNFGAAYAKAEAGAFGALPTEGTVFVTVANRDKRTLILPIQRLASMGYKILATEGTAGMLRRNGIDCEVVLKASDIREGVEGKSIVDRIREGEVDLILNTPAGSAGARHDGYDIRAAAVTVGVPLITTVQGVTAAVQGIEALREGVVSVRALQELDHAVKA

SEQ ID NO: 2 - DNA, 4529 bp, unidentified
  misc_feature 1..4529: note = carAB
  source 1..4529: mol_type = genomic DNA
gtgagtaaagacaccaccacctaccagggagtcaccgagatcggatccgttccggcatacctggttcttgcagacggacgtaccttcaccggatttggctttggagctatcggcaccacccttggtgaggcagtgttcaccaccgccatgaccggttaccaagaaaccatgaccgatccttcctatcaccgccagattgttgtggctaccgcaccacagatcggtaacaccggctggaacgatgaggacaacgagtcccgcgacggcaagatttgggttgcaggccttgttatccgcgacctcgcagcacgtgtgtccaactggcgcgccaccacctccttgcagcaggaaatggcagaccaaggcatcgtcggcatcggcggaatcgacacccgcgcactggttcgccacctgcgcaacgaaggttccatcgcagcgggcatcttctccggcgctgacgcacagcgcccagttgaagaactcgtagagatcgtcaagaatcagccagcaatgaccggcgcaaacctctccgttgaggtctctgctgatgaaacctacgtcatcgaagctgagggcgaagagcgccacaccgtcgtggcctacgacctgggcattaagcaaaacaccccacgtcgtttctctgcacgcggtgttcgcaccgtcatcgtgcctgctgaaaccccattggaggacatcaagcagtacaacccatcaggcgtgtttatctccaatggccctggcgaccctgcagcagcagacgtcatggttgatatcgtccgcgaagttctggaagccgacattccattctttggcatctgcttcggcaaccagatcctcggccgcgcattcggcatggagacctacaagctgaagttcggccaccgcggcatcaacgttccagtgaagaaccacatcaccggcaagatcgacatcaccgcccagaaccacggcttcgcactcaagggtgaagcaggccaggaattcgagacagatttcggcactgcgattgtcacccacacctgccttaacgacggcgtcgttgaaggtgttgcgctgaagtccggacgcgcatactccgttcagtaccacccagaggccgctgccggcccaaatgatgcaagccccctgtttgaccagtttgttgagctgatggatgcagacgctcagaagaaaggcgcataaataacatgccaaagcgttcagatattaaccacgtcctcgtcatcggttccggccccatcgtcattggccaggcatgtgaattcgactactccggcacccaggcttgccgcgtgctgaaggaagagggactgcgcgtcaccctcatcaactccaacccagcaacgatcatgaccgacccagaaatggctgaccacacctacgtggagccaatcgagccggaatacatcgacaagattttcgctaaggagatcgagcagggccacccaatcgacgccgtcctggcaacccttggtggccagactgcacttaacgcagctatccagctggatcgcctcggcatcctggaaaagtacggcgttgaactcatcggtgcagacatcgatgccattgagcgcggcgaagatcgccagaagttcaaggatattgtcaccaccatcggtggcgaatccgcgcgttcccgcgtctgccacaacatggacgaagtccatgagactgtcgcagaacttggccttccagtagtcgtgcgtccatccttcactatgggtggcctgggctccggtcttgcatacaacaccgaagaccttgagcgcatcgcaggtggcggacttgctgcatctcctgaagcaaacgtcttgatcgaagaatccatccttggttggaaggaattcgagctcgagctcatgcgcgataccgcagacaacgttgtggttatctgctccattgaaaacgtcgacgcactgggcgtgcacaccggcgactctgtcaccgtggcacctgccctgaccctgactgaccgtgaattccagaagatgcgcgatcagggtatcgccatcatccgcgaggtcggcgtggacaccggtggatgtaacatccagttcgctatcaacccagttgatggccgcatcatcaccattgagatgaacccacgtgtgtctcgttcctccgcgctggcatccaaggcaacgggcttcccaattgccaagatggctgccaagctggctatcggatacaccctggatgagatcaccaacgacatcactggtgaaaccccagctgcgtttgagcccaccatcgactacgtcgtggtcaaggccccacgctttgctttcgagaagtttgtcggcgctgatgacactttgaccaccaccatgaagtccgtcggtgaggtcatgtccctgggccgtaactacattgcagcactgaacaaggcactgcgttccctggaaaccaagcagcagggtttctggaccaagcctgatgagttcttcgcaggggagcgcgctaccgataaggcagctgttctggaagatctcaagcgcccaaccgaaggccgcctctacgacgttgagctggcaatgcgccttggcgcaagcgtggaagaactctacgaagcatcttctattgatccttggttcctcgccgagcttgaagctctcgtgcagttccgccagaagctcgttgacgcaccattcctcaacgaagatctcctgcgcgaagcaaagttcatgggtctgtccgacctgcagatcgcagcccttcgcccagagttcgctggcgaagacggcgtacgcaccttgcgtctgtccctaggcatccgcccagtattcaagactgtggatacctgtgcagcagagtttgaagctaagactccgtaccactactccgcatacgagctggatccagcagctgagtctgaggtcgcaccacagactgagcgtgaaaaggtcctgatcttgggctccggtccaaaccgcatcggccagggcatcgagttcgactattcctgtgttcacgcagctcttgagctctcccgcgtcggctacgaaactgtcatggtcaactgcaacccagagaccgtgtccaccgactacgacaccgctgaccgcctgtacttcgagccactgaccttcgaagacgtcatggaggtctaccacgctgaggcgcagtccggcaccgtcgcaggtgttatcgtccagcttggtggccagactcctctgggcttggcagatcgtttgaagaaggctggcgtccctgtcattggtacctccccagaggcaatcgacatggctgaggaccgtggcgagttcggtgcactgctgaaccgcgagcagcttcctgctccagcattcggcaccgcaacctctttcgaagaggctcgcacagtagccgatgagatcagctacccagtgctggttcgcccttcctacgtcttgggtggccgtggcatggagattgtctacgatgaggcttccctcgaggattacatcaaccgcgcaactgagttgtcttctgaccacccagtgctggttgaccgcttcctggacaacgctattgagatcgacgtcgacgcactgtgcgacggcgacgaagtctacctggcgggcgtcatggaacacatcgaggaagccggcattcactccggtgactccgcatgtgcacttcctccaatgactttgggcgcacaggacatcgagaaggtccgcgaagcaaccaagaagctggctctgggcatcggcgtacagggcctgatgaacgtccagtacgcactcaaggacgacatcctctacgtcatcgaggcaaacccacgtgcatcccgcaccgtgccgttcgtctccaaggcaacgggcgtcaacctggccaaggcagcatcccgtatcgcagtgggcgccaccatcaaggatctccaagatgagggcatgattcctaccgagtacgacggcggctccttgccactggacgctccaatcgctgtgaaggaagcagtgttgccgttcaaccgcttccgtcgcccagatggaaagaccctggacaccctgctttccccagagatgaagtccactggcgaggtcatgggcttggccaacaacttcggcgctgcatatgcaaaggctgaagctggcgcgtttggtgcattgccaaccgaaggcaccgtcttcgtgaccgtggctaaccgcgacaagcgcaccctgatcctgccaatccagcgcctggcgtcgatgggctacaagatcctcgccaccgaaggcaccgcaggcatgctgcgccgcaacggcattgattgtgaagttgtgctcaaggcttccgacatccgcgaaggtgtagagggcaagtccatcgtggatcgtatccgcgaaggcgaagttgacctcatcctcaacaccccagctggttctgctggcgctcgccacgatggctacgatatccgcgcagcagcagtgaccgtgggtgttccactgatcaccactgtccagggtgtcaccgcagctgtccagggcattgaggccctgcgtgagggcgttgtcagcgtccgcgcgctgcaggaactcgaccacgcagtcaaggcttaa

SEQ ID NO: 3 - protein, 1113 aa, synthetic construct
  REGION 1..1113: note = CarB(E799A) AA
MPKRSDINHVLVIGSGPIVIGQACEFDYSGTQACRVLKEEGLRVTLINSNPATIMTDPEMADHTYVEPIEPEYIDKIFAKEIEQGHPIDAVLATLGGQTALNAAIQLDRLGILEKYGVELIGADIDAIERGEDRQKFKDIVTTIGGESARSRVCHNMDEVHETVAELGLPVVVRPSFTMGGLGSGLAYNTEDLERIAGGGLAASPEANVLIEESILGWKEFELELMRDTADNVVVICSIENVDALGVHTGDSVTVAPALTLTDREFQKMRDQGIAIIREVGVDTGGCNIQFAINPVDGRIITIEMNPRVSRSSALASKATGFPIAKMAAKLAIGYTLDEITNDITGETPAAFEPTIDYVVVKAPRFAFEKFVGADDTLTTTMKSVGEVMSLGRNYIAALNKALRSLETKQQGFWTKPDEFFAGERATDKAAVLEDLKRPTEGRLYDVELAMRLGASVEELYEASSIDPWFLAELEALVQFRQKLVDAPFLNEDLLREAKFMGLSDLQIAALRPEFAGEDGVRTLRLSLGIRPVFKTVDTCAAEFEAKTPYHYSAYELDPAAESEVAPQTEREKVLILGSGPNRIGQGIEFDYSCVHAALELSRVGYETVMVNCNPETVSTDYDTADRLYFEPLTFEDVMEVYHAEAQSGTVAGVIVQLGGQTPLGLADRLKKAGVPVIGTSPEAIDMAEDRGEFGALLNREQLPAPAFGTATSFEEARTVADEISYPVLVRPSYVLGGRGMEIVYDEASLEDYINRATELSSDHPVLVDRFLDNAIEIDVDALCDGDEVYLAGVMEHIAEAGIHSGDSACALPPMTLGAQDIEKVREATKKLALGIGVQGLMNVQYALKDDILYVIEANPRASRTVPFVSKATGVNLAKAASRIAVGATIKDLQDEGMIPTEYDGGSLPLDAPIAVKEAVLPFNRFRRPDGKTLDTLLSPEMKSTGEVMGLANNFGAAYAKAEAGAFGALPTEGTVFVTVANRDKRTLILPIQRLASMGYKILATEGTAGMLRRNGIDCEVVLKASDIREGVEGKSIVDRIREGEVDLILNTPAGSAGARHDGYDIRAAAVTVGVPLITTVQGVTAAVQGIEALREGVVSVRALQELDHAVKA

SEQ ID NO: 4 - DNA, 3342 bp, synthetic construct
  misc_feature 1..3342: note = CarB(E799A) NT
  source 1..3342: mol_type = other DNA
atgccaaagcgttcagatattaaccacgtcctcgtcatcggttccggccccatcgtcattggccaggcatgtgaattcgactactccggcacccaggcttgccgcgtgctgaaggaagagggactgcgcgtcaccctcatcaactccaacccagcaacgatcatgaccgacccagaaatggctgaccacacctacgtggagccaatcgagccggaatacatcgacaagattttcgctaaggagatcgagcagggccacccaatcgacgccgtcctggcaacccttggtggccagactgcacttaacgcagctatccagctggatcgcctcggcatcctggaaaagtacggcgttgaactcatcggtgcagacatcgatgccattgagcgcggcgaagatcgccagaagttcaaggatattgtcaccaccatcggtggcgaatccgcgcgttcccgcgtctgccacaacatggacgaagtccatgagactgtcgcagaacttggccttccagtagtcgtgcgtccatccttcactatgggtggcctgggctccggtcttgcatacaacaccgaagaccttgagcgcatcgcaggtggcggacttgctgcatctcctgaagcaaacgtcttgatcgaagaatccatccttggttggaaggaattcgagctcgagctcatgcgcgataccgcagacaacgttgtggttatctgctccattgaaaacgtcgacgcactgggcgtgcacaccggcgactctgtcaccgtggcacctgccctgaccctgactgaccgtgaattccagaagatgcgcgatcagggtatcgccatcatccgcgaggtcggcgtggacaccggtggatgtaacatccagttcgctatcaacccagttgatggccgcatcatcaccattgagatgaacccacgtgtgtctcgttcctccgcgctggcatccaaggcaacgggcttcccaattgccaagatggctgccaagctggctatcggatacaccctggatgagatcaccaacgacatcactggtgaaaccccagctgcgtttgagcccaccatcgactacgtcgtggtcaaggccccacgctttgctttcgagaagtttgtcggcgctgatgacactttgaccaccaccatgaagtccgtcggtgaggtcatgtccctgggccgtaactacattgcagcactgaacaaggcactgcgttccctggaaaccaagcagcagggtttctggaccaagcctgatgagttcttcgcaggggagcgcgctaccgataaggcagctgttctggaagatctcaagcgcccaaccgaaggccgcctctacgacgttgagctggcaatgcgccttggcgcaagcgtggaagaactctacgaagcatcttctattgatccttggttcctcgccgagcttgaagctctcgtgcagttccgccagaagctcgttgacgcaccattcctcaacgaagatctcctgcgcgaagcaaagttcatgggtctgtccgacctgcagatcgcagcccttcgcccagagttcgctggcgaagacggcgtacgcaccttgcgtctgtccctaggcatccgcccagtattcaagactgtggatacctgtgcagcagagtttgaagctaagactccgtaccactactccgcatacgagctggatccagcagctgagtctgaggtcgcaccacagactgagcgtgaaaaggtcctgatcttgggctccggtccaaaccgcatcggccagggcatcgagttcgactattcctgtgttcacgcagctcttgagctctcccgcgtcggctacgaaactgtcatggtcaactgcaacccagagaccgtgtccaccgactacgacaccgctgaccgcctgtacttcgagccactgaccttcgaagacgtcatggaggtctaccacgctgaggcgcagtccggcaccgtcgcaggtgttatcgtccagcttggtggccagactcctctgggcttggcagatcgtttgaagaaggctggcgtccctgtcattggtacctccccagaggcaatcgacatggctgaggaccgtggcgagttcggtgcactgctgaaccgcgagcagcttcctgctccagcattcggcaccgcaacctctttcgaagaggctcgcacagtagccgatgagatcagctacccagtgctggttcgcccttcctacgtcttgggtggccgtggcatggagattgtctacgatgaggcttccctcgaggattacatcaaccgcgcaactgagttgtcttctgaccacccagtgctggttgaccgcttcctggacaacgctattgagatcgacgtcgacgcactgtgcgacggcgacgaagtctacctggcgggcgtcatggaacacatcgcagaagccggcattcactccggtgactccgcatgtgcacttcctccaatgactttgggcgcacaggacatcgagaaggtccgcgaagcaaccaagaagctggctctgggcatcggcgtacagggcctgatgaacgtccagtacgcactcaaggacgacatcctctacgtcatcgaggcaaacccacgtgcatcccgcaccgtgccgttcgtctccaaggcaacgggcgtcaacctggccaaggcagcatcccgtatcgcagtgggcgccaccatcaaggatctccaagatgagggcatgattcctaccgagtacgacggcggctccttgccactggacgctccaatcgctgtgaaggaagcagtgttgccgttcaaccgcttccgtcgcccagatggaaagaccctggacaccctgctttccccagagatgaagtccactggcgaggtcatgggcttggccaacaacttcggcgctgcatatgcaaaggctgaagctggcgcgtttggtgcattgccaaccgaaggcaccgtcttcgtgaccgtggctaaccgcgacaagcgcaccctgatcctgccaatccagcgcctggcgtcgatgggctacaagatcctcgccaccgaaggcaccgcaggcatgctgcgccgcaacggcattgattgtgaagttgtgctcaaggcttccgacatccgcgaaggtgtagagggcaagtccatcgtggatcgtatccgcgaaggcgaagttgacctcatcctcaacaccccagctggttctgctggcgctcgccacgatggctacgatatccgcgcagcagcagtgaccgtgggtgttccactgatcaccactgtccagggtgtcaccgcagctgtccagggcattgaggccctgcgtgagggcgttgtcagcgtccgcgcgctgcaggaactcgaccacgcagtcaaggcttaa

SEQ ID NO: 5 - protein, 1113 aa, synthetic construct
  REGION 1..1113: note = CarB(E799I) AA
MPKRSDINHVLVIGSGPIVIGQACEFDYSGTQACRVLKEEGLRVTLINSNPATIMTDPEMADHTYVEPIEPEYIDKIFAKEIEQGHPIDAVLATLGGQTALNAAIQLDRLGILEKYGVELIGADIDAIERGEDRQKFKDIVTTIGGESARSRVCHNMDEVHETVAELGLPVVVRPSFTMGGLGSGLAYNTEDLERIAGGGLAASPEANVLIEESILGWKEFELELMRDTADNVVVICSIENVDALGVHTGDSVTVAPALTLTDREFQKMRDQGIAIIREVGVDTGGCNIQFAINPVDGRIITIEMNPRVSRSSALASKATGFPIAKMAAKLAIGYTLDEITNDITGETPAAFEPTIDYVVVKAPRFAFEKFVGADDTLTTTMKSVGEVMSLGRNYIAALNKALRSLETKQQGFWTKPDEFFAGERATDKAAVLEDLKRPTEGRLYDVELAMRLGASVEELYEASSIDPWFLAELEALVQFRQKLVDAPFLNEDLLREAKFMGLSDLQIAALRPEFAGEDGVRTLRLSLGIRPVFKTVDTCAAEFEAKTPYHYSAYELDPAAESEVAPQTEREKVLILGSGPNRIGQGIEFDYSCVHAALELSRVGYETVMVNCNPETVSTDYDTADRLYFEPLTFEDVMEVYHAEAQSGTVAGVIVQLGGQTPLGLADRLKKAGVPVIGTSPEAIDMAEDRGEFGALLNREQLPAPAFGTATSFEEARTVADEISYPVLVRPSYVLGGRGMEIVYDEASLEDYINRATELSSDHPVLVDRFLDNAIEIDVDALCDGDEVYLAGVMEHIIEAGIHSGDSACALPPMTLGAQDIEKVREATKKLALGIGVQGLMNVQYALKDDILYVIEANPRASRTVPFVSKATGVNLAKAASRIAVGATIKDLQDEGMIPTEYDGGSLPLDAPIAVKEAVLPFNRFRRPDGKTLDTLLSPEMKSTGEVMGLANNFGAAYAKAEAGAFGALPTEGTVFVTVANRDKRTLILPIQRLASMGYKILATEGTAGMLRRNGIDCEVVLKASDIREGVEGKSIVDRIREGEVDLILNTPAGSAGARHDGYDIRAAAVTVGVPLITTVQGVTAAVQGIEALREGVVSVRALQELDHAVKA

SEQ ID NO: 6 - DNA, 3342 bp, synthetic construct
  misc_feature 1..3342: note = CarB(E799I) NT
  source 1..3342: mol_type = other DNA
atgccaaagcgttcagatattaaccacgtcctcgtcatcggttccggccccatcgtcattggccaggcatgtgaattcgactactccggcacccaggcttgccgcgtgctgaaggaagagggactgcgcgtcaccctcatcaactccaacccagcaacgatcatgaccgacccagaaatggctgaccacacctacgtggagccaatcgagccggaatacatcgacaagattttcgctaaggagatcgagcagggccacccaatcgacgccgtcctggcaacccttggtggccagactgcacttaacgcagctatccagctggatcgcctcggcatcctggaaaagtacggcgttgaactcatcggtgcagacatcgatgccattgagcgcggcgaagatcgccagaagttcaaggatattgtcaccaccatcggtggcgaatccgcgcgttcccgcgtctgccacaacatggacgaagtccatgagactgtcgcagaacttggccttccagtagtcgtgcgtccatccttcactatgggtggcctgggctccggtcttgcatacaacaccgaagaccttgagcgcatcgcaggtggcggacttgctgcatctcctgaagcaaacgtcttgatcgaagaatccatccttggttggaaggaattcgagctcgagctcatgcgcgataccgcagacaacgttgtggttatctgctccattgaaaacgtcgacgcactgggcgtgcacaccggcgactctgtcaccgtggcacctgccctgaccctgactgaccgtgaattccagaagatgcgcgatcagggtatcgccatcatccgcgaggtcggcgtggacaccggtggatgtaacatccagttcgctatcaacccagttgatggccgcatcatcaccattgagatgaacccacgtgtgtctcgttcctccgcgctggcatccaaggcaacgggcttcccaattgccaagatggctgccaagctggctatcggatacaccctggatgagatcaccaacgacatcactggtgaaaccccagctgcgtttgagcccaccatcgactacgtcgtggtcaaggccccacgctttgctttcgagaagtttgtcggcgctgatgacactttgaccaccaccatgaagtccgtcggtgaggtcatgtccctgggccgtaactacattgcagcactgaacaaggcactgcgttccctggaaaccaagcagcagggtttctggaccaagcctgatgagttcttcgcaggggagcgcgctaccgataaggcagctgttctggaagatctcaagcgcccaaccgaaggccgcctctacgacgttgagctggcaatgcgccttggcgcaagcgtggaagaactctacgaagcatcttctattgatccttggttcctcgccgagcttgaagctctcgtgcagttccgccagaagctcgttgacgcaccattcctcaacgaagatctcctgcgcgaagcaaagttcatgggtctgtccgacctgcagatcgcagcccttcgcccagagttcgctggcgaagacggcgtacgcaccttgcgtctgtccctaggcatccgcccagtattcaagactgtggatacctgtgcagcagagtttgaagctaagactccgtaccactactccgcatacgagctggatccagcagctgagtctgaggtcgcaccacagactgagcgtgaaaaggtcctgatcttgggctccggtccaaaccgcatcggccagggcatcgagttcgactattcctgtgttcacgcagctcttgagctctcccgcgtcggctacgaaactgtcatggtcaactgcaacccagagaccgtgtccaccgactacgacaccgctgaccgcctgtacttcgagccactgaccttcgaagacgtcatggaggtctaccacgctgaggcgcagtccggcaccgtcgcaggtgttatcgtccagcttggtggccagactcctctgggcttggcagatcgtttgaagaaggctggcgtccctgtcattggtacctccccagaggcaatcgacatggctgaggaccgtggcgagttcggtgcactgctgaaccgcgagcagcttcctgctccagcattcggcaccgcaacctctttcgaagaggctcgcacagtagccgatgagatcagctacccagtgctggttcgcccttcctacgtcttgggtggccgtggcatggagattgtctacgatgaggcttccctcgaggattacatcaaccgcgcaactgagttgtcttctgaccacccagtgctggttgaccgcttcctggacaacgctattgagatcgacgtcgacgcactgtgcgacggcgacgaagtctacctggcgggcgtcatggaacacatcatcgaagccggcattcactccggtgactccgcatgtgcacttcctccaatgactttgggcgcacaggacatcgagaaggtccgcgaagcaaccaagaagctggctctgggcatcggcgtacagggcctgatgaacgtccagtacgcactcaaggacgacatcctctacgtcatcgaggcaaacccacgtgcatcccgcaccgtgccgttcgtctccaaggcaacgggcgtcaacctggccaaggcagcatcccgtatcgcagtgggcgccaccatcaaggatctccaagatgagggcatgattcctaccgagtacgacggcggctccttgccactggacgctccaatcgctgtgaaggaagcagtgttgccgttcaaccgcttccgtcgcccagatggaaagaccctggacaccctgctttccccagagatgaagtccactggcgaggtcatgggcttggccaacaacttcggcgctgcatatgcaaaggctgaagctggcgcgtttggtgcattgccaaccgaaggcaccgtcttcgtgaccgtggctaaccgcgacaagcgcaccctgatcctgccaatccagcgcctggcgtcgatgggctacaagatcctcgccaccgaaggcaccgcaggcatgctgcgccgcaacggcattgattgtgaagttgtgctcaaggcttccgacatccgcgaaggtgtagagggcaagtccatcgtggatcgtatccgcgaaggcgaagttgacctcatcctcaacaccccagctggttctgctggcgctcgccacgatggctacgatatccgcgcagcagcagtgaccgtgggtgttccactgatcaccactgtccagggtgtcaccgcagctgtccagggcattgaggccctgcgtgagggcgttgtcagcgtccgcgcgctgcaggaactcgaccacgcagtcaaggcttaa

SEQ ID NO: 7 - protein, 1113 aa, synthetic construct
  REGION 1..1113: note = CarB(E799L) AA
MPKRSDINHVLVIGSGPIVIGQACEFDYSGTQACRVLKEEGLRVTLINSNPATIMTDPEMADHTYVEPIEPEYIDKIFAKEIEQGHPIDAVLATLGGQTALNAAIQLDRLGILEKYGVELIGADIDAIERGEDRQKFKDIVTTIGGESARSRVCHNMDEVHETVAELGLPVVVRPSFTMGGLGSGLAYNTEDLERIAGGGLAASPEANVLIEESILGWKEFELELMRDTADNVVVICSIENVDALGVHTGDSVTVAPALTLTDREFQKMRDQGIAIIREVGVDTGGCNIQFAINPVDGRIITIEMNPRVSRSSALASKATGFPIAKMAAKLAIGYTLDEITNDITGETPAAFEPTIDYVVVKAPRFAFEKFVGADDTLTTTMKSVGEVMSLGRNYIAALNKALRSLETKQQGFWTKPDEFFAGERATDKAAVLEDLKRPTEGRLYDVELAMRLGASVEELYEASSIDPWFLAELEALVQFRQKLVDAPFLNEDLLREAKFMGLSDLQIAALRPEFAGEDGVRTLRLSLGIRPVFKTVDTCAAEFEAKTPYHYSAYELDPAAESEVAPQTEREKVLILGSGPNRIGQGIEFDYSCVHAALELSRVGYETVMVNCNPETVSTDYDTADRLYFEPLTFEDVMEVYHAEAQSGTVAGVIVQLGGQTPLGLADRLKKAGVPVIGTSPEAIDMAEDRGEFGALLNREQLPAPAFGTATSFEEARTVADEISYPVLVRPSYVLGGRGMEIVYDEASLEDYINRATELSSDHPVLVDRFLDNAIEIDVDALCDGDEVYLAGVMEHILEAGIHSGDSACALPPMTLGAQDIEKVREATKKLALGIGVQGLMNVQYALKDDILYVIEANPRASRTVPFVSKATGVNLAKAASRIAVGATIKDLQDEGMIPTEYDGGSLPLDAPIAVKEAVLPFNRFRRPDGKTLDTLLSPEMKSTGEVMGLANNFGAAYAKAEAGAFGALPTEGTVFVTVANRDKRTLILPIQRLASMGYKILATEGTAGMLRRNGIDCEVVLKASDIREGVEGKSIVDRIREGEVDLILNTPAGSAGARHDGYDIRAAAVTVGVPLITTVQGVTAAVQGIEALREGVVSVRALQELDHAVKA

SEQ ID NO: 8 - DNA, 3342 bp, synthetic construct
  misc_feature 1..3342: note = CarB(E799L) NT
  source 1..3342: mol_type = other DNA
atgccaaagcgttcagatattaaccacgtcctcgtcatcggttccggccccatcgtcattggccaggcatgtgaattcgactactccggcacccaggcttgccgcgtgctgaaggaagagggactgcgcgtcaccctcatcaactccaacccagcaacgatcatgaccgacccagaaatggctgaccacacctacgtggagccaatcgagccggaatacatcgacaagattttcgctaaggagatcgagcagggccacccaatcgacgccgtcctggcaacccttggtggccagactgcacttaacgcagctatccagctggatcgcctcggcatcctggaaaagtacggcgttgaactcatcggtgcagacatcgatgccattgagcgcggcgaagatcgccagaagttcaaggatattgtcaccaccatcggtggcgaatccgcgcgttcccgcgtctgccacaacatggacgaagtccatgagactgtcgcagaacttggccttccagtagtcgtgcgtccatccttcactatgggtggcctgggctccggtcttgcatacaacaccgaagaccttgagcgcatcgcaggtggcggacttgctgcatctcctgaagcaaacgtcttgatcgaagaatccatccttggttggaaggaattcgagctcgagctcatgcgcgataccgcagacaacgttgtggttatctgctccattgaaaacgtcgacgcactgggcgtgcacaccggcgactctgtcaccgtggcacctgccctgaccctgactgaccgtgaattccagaagatgcgcgatcagggtatcgccatcatccgcgaggtcggcgtggacaccggtggatgtaacatccagttcgctatcaacccagttgatggccgcatcatcaccattgagatgaacccacgtgtgtctcgttcctccgcgctggcatccaaggcaacgggcttcccaattgccaagatggctgccaagctggctatcggatacaccctggatgagatcaccaacgacatcactggtgaaaccccagctgcgtttgagcccaccatcgactacgtcgtggtcaaggccccacgctttgctttcgagaagtttgtcggcgctgatgacactttgaccaccaccatgaagtccgtcggtgaggtcatgtccctgggccgtaactacattgcagcactgaacaaggcactgcgttccctggaaaccaagcagcagggtttctggaccaagcctgatgagttcttcgcaggggagcgcgctaccgataaggcagctgttctggaagatctcaagcgcccaaccgaaggccgcctctacgacgttgagctggcaatgcgccttggcgcaagcgtggaagaactctacgaagcatcttctattgatccttggttcctcgccgagcttgaagctctcgtgcagttccgccagaagctcgttgacgcaccattcctcaacgaagatctcctgcgcgaagcaaagttcatgggtctgtccgacctgcagatcgcagcccttcgcccagagttcgctggcgaagacggcgtacgcaccttgcgtctgtccctaggcatccgcccagtattcaagactgtggatacctgtgcagcagagtttgaagctaagactccgtaccactactccgcatacgagctggatccagcagctgagtctgaggtcgcaccacagactgagcgtgaaaaggtcctgatcttgggctccggtccaaaccgcatcggccagggcatcgagttcgactattcctgtgttcacgcagctcttgagctctcccgcgtcggctacgaaactgtcatggtcaactgcaacccagagaccgtgtccaccgactacgacaccgctgaccgcctgtacttcgagccactgaccttcgaagacgtcatggaggtctaccacgctgaggcgcagtccggcaccgtcgcaggtgttatcgtccagcttggtggccagactcctctgggcttggcagatcgtttgaagaaggctggcgtccctgtcattggtacctccccagaggcaatcgacatggctgaggaccgtggcgagttcggtgcactgctgaaccgcgagcagcttcctgctccagcattcggcaccgcaacctctttcgaagaggctcgcacagtagccgatgagatcagctacccagtgctggttcgcccttcctacgtcttgggtggccgtggcatggagattgtctacgatgaggcttccctcgaggattacatcaaccgcgcaactgagttgtcttctgaccacccagtgctggttgaccgcttcctggacaacgctattgagatcgacgtcgacgcactgtgcgacggcgacgaagtctacctggcgggcgtcatggaacacatcctcgaagccggcattcactccggtgactccgcatgtgcacttcctccaatgactttgggcgcacaggacatcgagaaggtccgcgaagcaaccaagaagctggctctgggcatcggcgtacagggcctgatgaacgtccagtacgcactcaaggacgacatcctctacgtcatcgaggcaaacccacgtgcatcccgcaccgtgccgttcgtctccaaggcaacgggcgtcaacctggccaaggcagcatcccgtatcgcagtgggcgccaccatcaaggatctccaagatgagggcatgattcctaccgagtacgacggcggctccttgccactggacgctccaatcgctgtgaaggaagcagtgttgccgttcaaccgcttccgtcgcccagatggaaagaccctggacaccctgctttccccagagatgaagtccactggcgaggtcatgggcttggccaacaacttcggcgctgcatatgcaaaggctgaagctggcgcgtttggtgcattgccaaccgaaggcaccgtcttcgtgaccgtggctaaccgcgacaagcgcaccctgatcctgccaatccagcgcctggcgtcgatgggctacaagatcctcgccaccgaaggcaccgcaggcatgctgcgccgcaacggcattgattgtgaagttgtgctcaaggcttccgacatccgcgaaggtgtagagggcaagtccatcgtggatcgtatccgcgaaggcgaagttgacctcatcctcaacaccccagctggttctgctggcgctcgccacgatggctacgatatccgcgcagcagcagtgaccgtgggtgttccactgatcaccactgtccagggtgtcaccgcagctgtccagggcattgaggccctgcgtgagggcgttgtcagcgtccgcgcgctgcaggaactcgaccacgcagtcaaggcttaa

SEQ ID NO: 9 - protein, 1113 aa, synthetic construct
  REGION 1..1113: note = CarB(E799V) AA
MPKRSDINHVLVIGSGPIVIGQACEFDYSGTQACRVLKEEGLRVTLINSNPATIMTDPEMADHTYVEPIEPEYIDKIFAKEIEQGHPIDAVLATLGGQTALNAAIQLDRLGILEKYGVELIGADIDAIERGEDRQKFKDIVTTIGGESARSRVCHNMDEVHETVAELGLPVVVRPSFTMGGLGSGLAYNTEDLERIAGGGLAASPEANVLIEESILGWKEFELELMRDTADNVVVICSIENVDALGVHTGDSVTVAPALTLTDREFQKMRDQGIAIIREVGVDTGGCNIQFAINPVDGRIITIEMNPRVSRSSALASKATGFPIAKMAAKLAIGYTLDEITNDITGETPAAFEPTIDYVVVKAPRFAFEKFVGADDTLTTTMKSVGEVMSLGRNYIAALNKALRSLETKQQGFWTKPDEFFAGERATDKAAVLEDLKRPTEGRLYDVELAMRLGASVEELYEASSIDPWFLAELEALVQFRQKLVDAPFLNEDLLREAKFMGLSDLQIAALRPEFAGEDGVRTLRLSLGIRPVFKTVDTCAAEFEAKTPYHYSAYELDPAAESEVAPQTEREKVLILGSGPNRIGQGIEFDYSCVHAALELSRVGYETVMVNCNPETVSTDYDTADRLYFEPLTFEDVMEVYHAEAQSGTVAGVIVQLGGQTPLGLADRLKKAGVPVIGTSPEAIDMAEDRGEFGALLNREQLPAPAFGTATSFEEARTVADEISYPVLVRPSYVLGGRGMEIVYDEASLEDYINRATELSSDHPVLVDRFLDNAIEIDVDALCDGDEVYLAGVMEHIVEAGIHSGDSACALPPMTLGAQDIEKVREATKKLALGIGVQGLMNVQYALKDDILYVIEANPRASRTVPFVSKATGVNLAKAASRIAVGATIKDLQDEGMIPTEYDGGSLPLDAPIAVKEAVLPFNRFRRPDGKTLDTLLSPEMKSTGEVMGLANNFGAAYAKAEAGAFGALPTEGTVFVTVANRDKRTLILPIQRLASMGYKILATEGTAGMLRRNGIDCEVVLKASDIREGVEGKSIVDRIREGEVDLILNTPAGSAGARHDGYDIRAAAVTVGVPLITTVQGVTAAVQGIEALREGVVSVRALQELDHAVKA

SEQ ID NO: 10 - DNA, 3342 bp, synthetic construct
  misc_feature 1..3342: note = CarB(E799V) NT
  source 1..3342: mol_type = other DNA
atgccaaagcgttcagatattaaccacgtcctcgtcatcggttccggccccatcgtcattggccaggcatgtgaattcgactactccggcacccaggcttgccgcgtgctgaaggaagagggactgcgcgtcaccctcatcaactccaacccagcaacgatcatgaccgacccagaaatggctgaccacacctacgtggagccaatcgagccggaatacatcgacaagattttcgctaaggagatcgagcagggccacccaatcgacgccgtcctggcaacccttggtggccagactgcacttaacgcagctatccagctggatcgcctcggcatcctggaaaagtacggcgttgaactcatcggtgcagacatcgatgccattgagcgcggcgaagatcgccagaagttcaaggatattgtcaccaccatcggtggcgaatccgcgcgttcccgcgtctgccacaacatggacgaagtccatgagactgtcgcagaacttggccttccagtagtcgtgcgtccatccttcactatgggtggcctgggctccggtcttgcatacaacaccgaagaccttgagcgcatcgcaggtggcggacttgctgcatctcctgaagcaaacgtcttgatcgaagaatccatccttggttggaaggaattcgagctcgagctcatgcgcgataccgcagacaacgttgtggttatctgctccattgaaaacgtcgacgcactgggcgtgcacaccggcgactctgtcaccgtggcacctgccctgaccctgactgaccgtgaattccagaagatgcgcgatcagggtatcgccatcatccgcgaggtcggcgtggacaccggtggatgtaacatccagttcgctatcaacccagttgatggccgcatcatcaccattgagatgaacccacgtgtgtctcgttcctccgcgctggcatccaaggcaacgggcttcccaattgccaagatggctgccaagctggctatcggatacaccctggatgagatcaccaacgacatcactggtgaaaccccagctgcgtttgagcccaccatcgactacgtcgtggtcaaggccccacgctttgctttcgagaagtttgtcggcgctgatgacactttgaccaccaccatgaagtccgtcggtgaggtcatgtccctgggccgtaactacattgcagcactgaacaaggcactgcgttccctggaaaccaagcagcagggtttctggaccaagcctgatgagttcttcgcaggggagcgcgctaccgataaggcagctgttctggaagatctcaagcgcccaaccgaaggccgcctctacgacgttgagctggcaatgcgccttggcgcaagcgtggaagaactctacgaagcatcttctattgatccttggttcctcgccgagcttgaagctctcgtgcagttccgccagaagctcgttgacgcaccattcctcaacgaagatctcctgcgcgaagcaaagttcatgggtctgtccgacctgcagatcgcagcccttcgcccagagttcgctggcgaagacggcgtacgcaccttgcgtctgtccctaggcatccgcccagtattcaagactgtggatacctgtgcagcagagtttgaagctaagactccgtaccactactccgcatacgagctggatccagcagctgagtctgaggtcgcaccacagactgagcgtgaaaaggtcctgatcttgggctccggtccaaaccgcatcggccagggcatcgagttcgactattcctgtgttcacgcagctcttgagctctcccgcgtcggctacgaaactgtcatggtcaactgcaacccagagaccgtgtccaccgactacgacaccgctgaccgcctgtacttcgagccactgaccttcgaagacgtcatggaggtctaccacgctgaggcgcagtccggcaccgtcgcaggtgttatcgtccagcttggtggccagactcctctgggcttggcagatcgtttgaagaaggctggcgtccctgtcattggtacctccccagaggcaatcgacatggctgaggaccgtggcgagttcggtgcactgctgaaccgcgagcagcttcctgctccagcattcggcaccgcaacctctttcgaagaggctcgcacagtagccgatgagatcagctacccagtgctggttcgcccttcctacgtcttgggtggccgtggcatggagattgtctacgatgaggcttccctcgaggattacatcaaccgcgcaactgagttgtcttctgaccacccagtgctggttgaccgcttcctggacaacgctattgagatcgacgtcgacgcactgtgcgacggcgacgaagtctacctggcgggcgtcatggaacacatcgtcgaagccggcattcactccggtgactccgcatgtgcacttcctccaatgactttgggcgcacaggacatcgagaaggtccgcgaagcaaccaagaagctggctctgggcatcggcgtacagggcctgatgaacgtccagtacgcactcaaggacgacatcctctacgtcatcgaggcaaacccacgtgcatcccgcaccgtgccgttcgtctccaaggcaacgggcgtcaacctggccaaggcagcatcccgtatcgcagtgggcgccaccatcaaggatctccaagatgagggcatgattcctaccgagtacgacggcggctccttgccactggacgctccaatcgctgtgaaggaagcagtgttgccgttcaaccgcttccgtcgcccagatggaaagaccctggacaccctgctttccccagagatgaagtccactggcgaggtcatgggcttggccaacaacttcggcgctgcatatgcaaaggctgaagctggcgcgtttggtgcattgccaaccgaaggcaccgtcttcgtgaccgtggctaaccgcgacaagcgcaccctgatcctgccaatccagcgcctggcgtcgatgggctacaagatcctcgccaccgaaggcaccgcaggcatgctgcgccgcaacggcattgattgtgaagttgtgctcaaggcttccgacatccgcgaaggtgtagagggcaagtccatcgtggatcgtatccgcgaaggcgaagttgacctcatcctcaacaccccagctggttctgctggcgctcgccacgatggctacgatatccgcgcagcagcagtgaccgtgggtgttccactgatcaccactgtccagggtgtcaccgcagctgtccagggcattgaggccctgcgtgagggcgttgtcagcgtccgcgcgctgcaggaactcgaccacgcagtcaaggcttaa

SEQ ID NO: 11 - protein, 1113 aa, synthetic construct
  REGION 1..1113: note = CarB(E918A) AA
MPKRSDINHVLVIGSGPIVIGQACEFDYSGTQACRVLKEEGLRVTLINSNPATIMTDPEMADHTYVEPIEPEYIDKIFAKEIEQGHPIDAVLATLGGQTALNAAIQLDRLGILEKYGVELIGADIDAIERGEDRQKFKDIVTTIGGESARSRVCHNMDEVHETVAELGLPVVVRPSFTMGGLGSGLAYNTEDLERIAGGGLAASPEANVLIEESILGWKEFELELMRDTADNVVVICSIENVDALGVHTGDSVTVAPALTLTDREFQKMRDQGIAIIREVGVDTGGCNIQFAINPVDGRIITIEMNPRVSRSSALASKATGFPIAKMAAKLAIGYTLDEITNDITGETPAAFEPTIDYVVVKAPRFAFEKFVGADDTLTTTMKSVGEVMSLGRNYIAALNKALRSLETKQQGFWTKPDEFFAGERATDKAAVLEDLKRPTEGRLYDVELAMRLGASVEELYEASSIDPWFLAELEALVQFRQKLVDAPFLNEDLLREAKFMGLSDLQIAALRPEFAGEDGVRTLRLSLGIRPVFKTVDTCAAEFEAKTPYHYSAYELDPAAESEVAPQTEREKVLILGSGPNRIGQGIEFDYSCVHAALELSRVGYETVMVNCNPETVSTDYDTADRLYFEPLTFEDVMEVYHAEAQSGTVAGVIVQLGGQTPLGLADRLKKAGVPVIGTSPEAIDMAEDRGEFGALLNREQLPAPAFGTATSFEEARTVADEISYPVLVRPSYVLGGRGMEIVYDEASLEDYINRATELSSDHPVLVDRFLDNAIEIDVDALCDGDEVYLAGVMEHIEEAGIHSGDSACALPPMTLGAQDIEKVREATKKLALGIGVQGLMNVQYALKDDILYVIEANPRASRTVPFVSKATGVNLAKAASRIAVGATIKDLQDEGMIPTEYDGGSLPLDAPIAVKAAVLPFNRFRRPDGKTLDTLLSPEMKSTGEVMGLANNFGAAYAKAEAGAFGALPTEGTVFVTVANRDKRTLILPIQRLASMGYKILATEGTAGMLRRNGIDCEVVLKASDIREGVEGKSIVDRIREGEVDLILNTPAGSAGARHDGYDIRAAAVTVGVPLITTVQGVTAAVQGIEALREGVVSVRALQELDHAVKA

SEQ ID NO: 12 - DNA, 3342 bp, synthetic construct
  misc_feature 1..3342: note = CarB(E918A) NT
  source 1..3342: mol_type = other DNA
atgccaaagcgttcagatattaaccacgtcctcgtcatcggttccggccccatcgtcattggccaggcatgtgaattcgactactccggcacccaggcttgccgcgtgctgaaggaagagggactgcgcgtcaccctcatcaactccaacccagcaacgatcatgaccgacccagaaatggctgaccacacctacgtggagccaatcgagccggaatacatcgacaagattttcgctaaggagatcgagcagggccacccaatcgacgccgtcctggcaacccttggtggccagactgcacttaacgcagctatccagctggatcgcctcggcatcctggaaaagtacggcgttgaactcatcggtgcagacatcgatgccattgagcgcggcgaagatcgccagaagttcaaggatattgtcaccaccatcggtggcgaatccgcgcgttcccgcgtctgccacaacatggacgaagtccatgagactgtcgcagaacttggccttccagtagtcgtgcgtccatccttcactatgggtggcctgggctccggtcttgcatacaacaccgaagaccttgagcgcatcgcaggtggcggacttgctgcatctcctgaagcaaacgtcttgatcgaagaatccatccttggttggaaggaattcgagctcgagctcatgcgcgataccgcagacaacgttgtggttatctgctccattgaaaacgtcgacgcactgggcgtgcacaccggcgactctgtcaccgtggcacctgccctgaccctgactgaccgtgaattccagaagatgcgcgatcagggtatcgccatcatccgcgaggtcggcgtggacaccggtggatgtaacatccagttcgctatcaacccagttgatggccgcatcatcaccattgagatgaacccacgtgtgtctcgttcctccgcgctggcatccaaggcaacgggcttcccaattgccaagatggctgccaagctggctatcggatacaccctggatgagatcaccaacgacatcactggtgaaaccccagctgcgtttgagcccaccatcgactacgtcgtggtcaaggccccacgctttgctttcgagaagtttgtcggcgctgatgacactttgaccaccaccatgaagtccgtcggtgaggtcatgtccctgggccgtaactacattgcagcactgaacaaggcactgcgttccctggaaaccaagcagcagggtttctggaccaagcctgatgagttcttcgcaggggagcgcgctaccgataaggcagctgttctggaagatctcaagcgcccaaccgaaggccgcctctacgacgttgagctggcaatgcgccttggcgcaagcgtggaagaactctacgaagcatcttctattgatccttggttcctcgccgagcttgaagctctcgtgcagttccgccagaagctcgttgacgcaccattcctcaacgaagatctcctgcgcgaagcaaagttcatgggtctgtccgacctgcagatcgcagcccttcgcccagagttcgctggcgaagacggcgtacgcaccttgcgtctgtccctaggcatccgcccagtattcaagactgtggatacctgtgcagcagagtttgaagctaagactccgtaccactactccgcatacgagctggatccagcagctgagtctgaggtcgcaccacagactgagcgtgaaaaggtcctgatcttgggctccggtccaaaccgcatcggccagggcatcgagttcgactattcctgtgttcacgcagctcttgagctctcccgcgtcggctacgaaactgtcatggtcaactgcaacccagagaccgtgtccaccgactacgacaccgctgaccgcctgtacttcgagccactgaccttcgaagacgtcatggaggtctaccacgctgaggcgcagtccggcaccgtcgcaggtgttatcgtccagcttggtggccagactcctctgggcttggcagatcgtttgaagaaggctggcgtccctgtcattggtacctccccagaggcaatcgacatggctgaggaccgtggcgagttcggtgcactgctgaaccgcgagcagcttcctgctccagcattcggcaccgcaacctctttcgaagaggctcgcacagtagccgatgagatcagctacccagtgctggttcgcccttcctacgtcttgggtggccgtggcatggagattgtctacgatgaggcttccctcgaggattacatcaaccgcgcaactgagttgtcttctgaccacccagtgctggttgaccgcttcctggacaacgctattgagatcgacgtcgacgcactgtgcgacggcgacgaagtctacctggcgggcgtcatggaacacatcgaggaagccggcattcactccggtgactccgcatgtgcacttcctccaatgactttgggcgcacaggacatcgagaaggtccgcgaagcaaccaagaagctggctctgggcatcggcgtacagggcctgatgaacgtccagtacgcactcaaggacgacatcctctacgtcatcgaggcaaacccacgtgcatcccgcaccgtgccgttcgtctccaaggcaacgggcgtcaacctggccaaggcagcatcccgtatcgcagtgggcgccaccatcaaggatctccaagatgagggcatgattcctaccgagtacgacggcggctccttgccactggacgctccaatcgctgtgaaggcagcagtgttgccgttcaaccgcttccgtcgcccagatggaaagaccctggacaccctgctttccccagagatgaagtccactggcgaggtcatgggcttggccaacaacttcggcgctgcatatgcaaaggctgaagctggcgcgtttggtgcattgccaaccgaaggcaccgtcttcgtgaccgtggctaaccgcgacaagcgcaccctgatcctgccaatccagcgcctggcgtcgatgggctacaagatcctcgccaccgaaggcaccgcaggcatgctgcgccgcaacggcattgattgtgaagttgtgctcaaggcttccgacatccgcgaaggtgtagagggcaagtccatcgtggatcgtatccgcgaaggcgaagttgacctcatcctcaacaccccagctggttctgctggcgctcgccacgatggctacgatatccgcgcagcagcagtgaccgtgggtgttccactgatcaccactgtccagggtgtcaccgcagctgtccagggcattgaggccctgcgtgagggcgttgtcagcgtccgcgcgctgcaggaactcgaccacgcagtcaaggcttaa

SEQ ID NO: 13 - protein, 1113 aa, synthetic construct
  REGION 1..1113: note = CarB(E918I) AA
MPKRSDINHVLVIGSGPIVIGQACEFDYSGTQACRVLKEEGLRVTLINSNPATIMTDPEMADHTYVEPIEPEYIDKIFAKEIEQGHPIDAVLATLGGQTALNAAIQLDRLGILEKYGVELIGADIDAIERGEDRQKFKDIVTTIGGESARSRVCHNMDEVHETVAELGLPVVVRPSFTMGGLGSGLAYNTEDLERIAGGGLAASPEANVLIEESILGWKEFELELMRDTADNVVVICSIENVDALGVHTGDSVTVAPALTLTDREFQKMRDQGIAIIREVGVDTGGCNIQFAINPVDGRIITIEMNPRVSRSSALASKATGFPIAKMAAKLAIGYTLDEITNDITGETPAAFEPTIDYVVVKAPRFAFEKFVGADDTLTTTMKSVGEVMSLGRNYIAALNKALRSLETKQQGFWTKPDEFFAGERATDKAAVLEDLKRPTEGRLYDVELAMRLGASVEELYEASSIDPWFLAELEALVQFRQKLVDAPFLNEDLLREAKFMGLSDLQIAALRPEFAGEDGVRTLRLSLGIRPVFKTVDTCAAEFEAKTPYHYSAYELDPAAESEVAPQTEREKVLILGSGPNRIGQGIEFDYSCVHAALELSRVGYETVMVNCNPETVSTDYDTADRLYFEPLTFEDVMEVYHAEAQSGTVAGVIVQLGGQTPLGLADRLKKAGVPVIGTSPEAIDMAEDRGEFGALLNREQLPAPAFGTATSFEEARTVADEISYPVLVRPSYVLGGRGMEIVYDEASLEDYINRATELSSDHPVLVDRFLDNAIEIDVDALCDGDEVYLAGVMEHIEEAGIHSGDSACALPPMTLGAQDIEKVREATKKLALGIGVQGLMNVQYALKDDILYVIEANPRASRTVPFVSKATGVNLAKAASRIAVGATIKDLQDEGMIPTEYDGGSLPLDAPIAVKIAVLPFNRFRRPDGKTLDTLLSPEMKSTGEVMGLANNFGAAYAKAEAGAFGALPTEGTVFVTVANRDKRTLILPIQRLASMGYKILATEGTAGMLRRNGIDCEVVLKASDIREGVEGKSIVDRIREGEVDLILNTPAGSAGARHDGYDIRAAAVTVGVPLITTVQGVTAAVQGIEALREGVVSVRALQELDHAVKA

SEQ ID NO: 14 - DNA, 3342 bp, synthetic construct
  misc_feature 1..3342: note = CarB(E918I) NT
  source 1..3342: mol_type = other DNA
atgccaaagcgttcagatattaaccacgtcctcgtcatcggttccggccccatcgtcattggccaggcatgtgaattcgactactccggcacccaggcttgccgcgtgctgaaggaagagggactgcgcgtcaccctcatcaactccaacccagcaacgatcatgaccgacccagaaatggctgaccacacctacgtggagccaatcgagccggaatacatcgacaagattttcgctaaggagatcgagcagggccacccaatcgacgccgtcctggcaacccttggtggccagactgcacttaacgcagctatccagctggatcgcctcggcatcctggaaaagtacggcgttgaactcatcggtgcagacatcgatgccattgagcgcggcgaagatcgccagaagttcaaggatattgtcaccaccatcggtggcgaatccgcgcgttcccgcgtctgccacaacatggacgaagtccatgagactgtcgcagaacttggccttccagtagtcgtgcgtccatccttcactatgggtggcctgggctccggtcttgcatacaacaccgaagaccttgagcgcatcgcaggtggcggacttgctgcatctcctgaagcaaacgtcttgatcgaagaatccatccttggttggaaggaattcgagctcgagctcatgcgcgataccgcagacaacgttgtggttatctgctccattgaaaacgtcgacgcactgggcgtgcacaccggcgactctgtcaccgtggcacctgccctgaccctgactgaccgtgaattccagaagatgcgcgatcagggtatcgccatcatccgcgaggtcggcgtggacaccggtggatgtaacatccagttcgctatcaacccagttgatggccgcatcatcaccattgagatgaacccacgtgtgtctcgttcctccgcgctggcatccaaggcaacgggcttcccaattgccaagatggctgccaagctggctatcggatacaccctggatgagatcaccaacgacatcactggtgaaaccccagctgcgtttgagcccaccatcgactacgtcgtggtcaaggccccacgctttgctttcgagaagtttgtcggcgctgatgacactttgaccaccaccatgaagtccgtcggtgaggtcatgtccctgggccgtaactacattgcagcactgaacaaggcactgcgttccctggaaaccaagcagcagggtttctggaccaagcctgatgagttcttcgcaggggagcgcgctaccgataaggcagctgttctggaagatctcaagcgcccaaccgaaggccgcctctacgacgttgagctggcaatgcgccttggcgcaagcgtggaagaactctacgaagcatcttctattgatccttggttcctcgccgagcttgaagctctcgtgcagttccgccagaagctcgttgacgcaccattcctcaacgaagatctcctgcgcgaagcaaagttcatgggtctgtccgacctgcagatcgcagcccttcgcccagagttcgctggcgaagacggcgtacgcaccttgcgtctgtccctaggcatccgcccagtattcaagactgtggatacctgtgcagcagagtttgaagctaagactccgtaccactactccgcatacgagctggatccagcagctgagtctgaggtcgcaccacagactgagcgtgaaaaggtcctgatcttgggctccggtccaaaccgcatcggccagggcatcgagttcgactattcctgtgttcacgcagctcttgagctctcccgcgtcggctacgaaactgtcatggtcaactgcaacccagagaccgtgtccaccgactacgacaccgctgaccgcctgtacttcgagccactgaccttcgaagacgtcatggaggtctaccacgctgaggcgcagtccggcaccgtcgcaggtgttatcgtccagcttggtggccagactcctctgggcttggcagatcgtttgaagaaggctggcgtccctgtcattggtacctccccagaggcaatcgacatggctgaggaccgtggcgagttcggtgcactgctgaaccgcgagcagcttcctgctccagcattcggcaccgcaacctctttcgaagaggctcgcacagtagccgatgagatcagctacccagtgctggttcgcccttcctacgtcttgggtggccgtggcatggagattgtctacgatgaggcttccctcgaggattacatcaaccgcgcaactgagttgtcttctgaccacccagtgctggttgaccgcttcctggacaacgctattgagatcgacgtcgacgcactgtgcgacggcgacgaagtctacctggcgggcgtcatggaacacatcgaggaagccggcattcactccggtgactccgcatgtgcacttcctccaatgactttgggcgcacaggacatcgagaaggtccgcgaagcaaccaagaagctggctctgggcatcggcgtacagggcctgatgaacgtccagtacgcactcaaggacgacatcctctacgtcatcgaggcaaacccacgtgcatcccgcaccgtgccgttcgtctccaaggcaacgggcgtcaacctggccaaggcagcatcccgtatcgcagtgggcgccaccatcaaggatctccaagatgagggcatgattcctaccgagtacgacggcggctccttgccactggacgctccaatcgctgtgaagatcgcagtgttgccgttcaaccgcttccgtcgcccagatggaaagaccctggacaccctgctttccccagagatgaagtccactggcgaggtcatgggcttggccaacaacttcggcgctgcatatgcaaaggctgaagctggcgcgtttggtgcattgccaaccgaaggcaccgtcttcgtgaccgtggctaaccgcgacaagcgcaccctgatcctgccaatccagcgcctggcgtcgatgggctacaagatcctcgccaccgaaggcaccgcaggcatgctgcgccgcaacggcattgattgtgaagttgtgctcaaggcttccgacatccgcgaaggtgtagagggcaagtccatcgtggatcgtatccgcgaaggcgaagttgacctcatcctcaacaccccagctggttctgctggcgctcgccacgatggctacgatatccgcgcagcagcagtgaccgtgggtgttccactgatcaccactgtccagggtgtcaccgcagctgtccagggcattgaggccctgcgtgagggcgttgtcagcgtccgcgcgctgcaggaactcgaccacgcagtcaaggcttaa

SEQ ID NO: 15 - protein, 1113 aa, synthetic construct
  REGION 1..1113: note = CarB(E918L) AA
MPKRSDINHVLVIGSGPIVIGQACEFDYSGTQACRVLKEEGLRVTLINSNPATIMTDPEMADHTYVEPIEPEYIDKIFAKEIEQGHPIDAVLATLGGQTALNAAIQLDRLGILEKYGVELIGADIDAIERGEDRQKFKDIVTTIGGESARSRVCHNMDEVHETVAELGLPVVVRPSFTMGGLGSGLAYNTEDLERIAGGGLAASPEANVLIEESILGWKEFELELMRDTADNVVVICSIENVDALGVHTGDSVTVAPALTLTDREFQKMRDQGIAIIREVGVDTGGCNIQFAINPVDGRIITIEMNPRVSRSSALASKATGFPIAKMAAKLAIGYTLDEITNDITGETPAAFEPTIDYVVVKAPRFAFEKFVGADDTLTTTMKSVGEVMSLGRNYIAALNKALRSLETKQQGFWTKPDEFFAGERATDKAAVLEDLKRPTEGRLYDVELAMRLGASVEELYEASSIDPWFLAELEALVQFRQKLVDAPFLNEDLLREAKFMGLSDLQIAALRPEFAGEDGVRTLRLSLGIRPVFKTVDTCAAEFEAKTPYHYSAYELDPAAESEVAPQTEREKVLILGSGPNRIGQGIEFDYSCVHAALELSRVGYETVMVNCNPETVSTDYDTADRLYFEPLTFEDVMEVYHAEAQSGTVAGVIVQLGGQTPLGLADRLKKAGVPVIGTSPEAIDMAEDRGEFGALLNREQLPAPAFGTATSFEEARTVADEISYPVLVRPSYVLGGRGMEIVYDEASLEDYINRATELSSDHPVLVDRFLDNAIEIDVDALCDGDEVYLAGVMEHIEEAGIHSGDSACALPPMTLGAQDIEKVREATKKLALGIGVQGLMNVQYALKDDILYVIEANPRASRTVPFVSKATGVNLAKAASRIAVGATIKDLQDEGMIPTEYDGGSLPLDAPIAVKLAVLPFNRFRRPDGKTLDTLLSPEMKSTGEVMGLANNFGAAYAKAEAGAFGALPTEGTVFVTVANRDKRTLILPIQRLASMGYKILATEGTAGMLRRNGIDCEVVLKASDIREGVEGKSIVDRIREGEVDLILNTPAGSAGARHDGYDIRAAAVTVGVPLITTVQGVTAAVQGIEALREGVVSVRALQELDHAVKA

SEQ ID NO: 16 - DNA, 3342 bp, synthetic construct
  misc_feature 1..3342: note = CarB(E918L) NT
  source 1..3342: mol_type = other DNA
atgccaaagcgttcagatattaaccacgtcctcgtcatcggttccggccccatcgtcattggccaggcatgtgaattcgactactccggcacccaggcttgccgcgtgctgaaggaagagggactgcgcgtcaccctcatcaactccaacccagcaacgatcatgaccgacccagaaatggctgaccacacctacgtggagccaatcgagccggaatacatcgacaagattttcgctaaggagatcgagcagggccacccaatcgacgccgtcctggcaacccttggtggccagactgcacttaacgcagctatccagctggatcgcctcggcatcctggaaaagtacggcgttgaactcatcggtgcagacatcgatgccattgagcgcggcgaagatcgccagaagttcaaggatattgtcaccaccatcggtggcgaatccgcgcgttcccgcgtctgccacaacatggacgaagtccatgagactgtcgcagaacttggccttccagtagtcgtgcgtccatccttcactatgggtggcctgggctccggtcttgcatacaacaccgaagaccttgagcgcatcgcaggtggcggacttgctgcatctcctgaagcaaacgtcttgatcgaagaatccatccttggttggaaggaattcgagctcgagctcatgcgcgataccgcagacaacgttgtggttatctgctccattgaaaacgtcgacgcactgggcgtgcacaccggcgactctgtcaccgtggcacctgccctgaccctgactgaccgtgaattccagaagatgcgcgatcagggtatcgccatcatccgcgaggtcggcgtggacaccggtggatgtaacatccagttcgctatcaacccagttgatggccgcatcatcaccattgagatgaacccacgtgtgtctcgttcctccgcgctggcatccaaggcaacgggcttcccaattgccaagatggctgccaagctggctatcggatacaccctggatgagatcaccaacgacatcactggtgaaaccccagctgcgtttgagcccaccatcgactacgtcgtggtcaaggccccacgctttgctttcgagaagtttgtcggcgctgatgacactttgaccaccaccatgaagtccgtcggtgaggtcatgtccctgggccgtaactacattgcagcactgaacaaggcactgcgttccctggaaaccaagcagcagggtttctggaccaagcctgatgagttcttcgcaggggagcgcgctaccgataaggcagctgttctggaagatctcaagcgcccaaccgaaggccgcctctacgacgttgagctggcaatgcgccttggcgcaagcgtggaagaactctacgaagcatcttctattgatccttggttcctcgccgagcttgaagctctcgtgcagttccgccagaagctcgttgacgcaccattcctcaacgaagatctcctgcgcgaagcaaagttcatgggtctgtccgacctgcagatcgcagcccttcgcccagagttcgctggcgaagacggcgtacgcaccttgcgtctgtccctaggcatccgcccagtattcaagactgtggatacctgtgcagcagagtttgaagctaagactccgtaccactactccgcatacgagctggatccagcagctgagtctgaggtcgcaccacagactgagcgtgaaaaggtcctgatcttgggctccggtccaaaccgcatcggccagggcatcgagttcgactattcctgtgttcacgcagctcttgagctctcccgcgtcggctacgaaactgtcatggtcaactgcaacccagagaccgtgtccaccgactacgacaccgctgaccgcctgtacttcgagccactgaccttcgaagacgtcatggaggtctaccacgctgaggcgcagtccggcaccgtcgcaggtgttatcgtccagcttggtggccagactcctctgggcttggcagatcgtttgaagaaggctggcgtccctgtcattggtacctccccagaggcaatcgacatggctgaggaccgtggcgagttcggtgcactgctgaaccgcgagcagcttcctgctccagcattcggcaccgcaacctctttcgaagaggctcgcacagtagccgatgagatcagctacccagtgctggttcgcccttcctacgtcttgggtggccgtggcatggagattgtctacgatgaggcttccctcgaggattacatcaaccgcgcaactgagttgtcttctgaccacccagtgctggttgaccgcttcctggacaacgctattgagatcgacgtcgacgcactgtgcgacggcgacgaagtctacctggcgggcgtcatggaacacatcgaggaagccggcattcactccggtgactccgcatgtgcacttcctccaatgactttgggcgcacaggacatcgagaaggtccgcgaagcaaccaagaagctggctctgggcatcggcgtacagggcctgatgaacgtccagtacgcactcaaggacgacatcctctacgtcatcgaggcaaacccacgtgcatcccgcaccgtgccgttcgtctccaaggcaacgggcgtcaacctggccaaggcagcatcccgtatcgcagtgggcgccaccatcaaggatctccaagatgagggcatgattcctaccgagtacgacggcggctccttgccactggacgctccaatcgctgtgaagctcgcagtgttgccgttcaaccgcttccgtcgcccagatggaaagaccctggacaccctgctttccccagagatgaagtccactggcgaggtcatgggcttggccaacaacttcggcgctgcatatgcaaaggctgaagctggcgcgtttggtgcattgccaaccgaaggcaccgtcttcgtgaccgtggctaaccgcgacaagcgcaccctgatcctgccaatccagcgcctggcgtcgatgggctacaagatcctcgccaccgaaggcaccgcaggcatgctgcgccgcaacggcattgattgtgaagttgtgctcaaggcttccgacatccgcgaaggtgtagagggcaagtccatcgtggatcgtatccgcgaaggcgaagttgacctcatcctcaacaccccagctggttctgctggcgctcgccacgatggctacgatatccgcgcagcagcagtgaccgtgggtgttccactgatcaccactgtccagggtgtcaccgcagctgtccagggcattgaggccctgcgtgagggcgttgtcagcgtccgcgcgctgcaggaactcgaccacgcagtcaaggcttaa

SEQ ID NO: 17 - protein, 1113 aa, synthetic construct
  REGION 1..1113: note = CarB(E918V) AA
MPKRSDINHVLVIGSGPIVIGQACEFDYSGTQACRVLKEEGLRVTLINSNPATIMTDPEMADHTYVEPIEPEYIDKIFAKEIEQGHPIDAVLATLGGQTALNAAIQLDRLGILEKYGVELIGADIDAIERGEDRQKFKDIVTTIGGESARSRVCHNMDEVHETVAELGLPVVVRPSFTMGGLGSGLAYNTEDLERIAGGGLAASPEANVLIEESILGWKEFELELMRDTADNVVVICSIENVDALGVHTGDSVTVAPALTLTDREFQKMRDQGIAIIREVGVDTGGCNIQFAINPVDGRIITIEMNPRVSRSSALASKATGFPIAKMAAKLAIGYTLDEITNDITGETPAAFEPTIDYVVVKAPRFAFEKFVGADDTLTTTMKSVGEVMSLGRNYIAALNKALRSLETKQQGFWTKPDEFFAGERATDKAAVLEDLKRPTEGRLYDVELAMRLGASVEELYEASSIDPWFLAELEALVQFRQKLVDAPFLNEDLLREAKFMGLSDLQIAALRPEFAGEDGVRTLRLSLGIRPVFKTVDTCAAEFEAKTPYHYSAYELDPAAESEVAPQTEREKVLILGSGPNRIGQGIEFDYSCVHAALELSRVGYETVMVNCNPETVSTDYDTADRLYFEPLTFEDVMEVYHAEAQSGTVAGVIVQLGGQTPLGLADRLKKAGVPVIGTSPEAIDMAEDRGEFGALLNREQLPAPAFGTATSFEEARTVADEISYPVLVRPSYVLGGRGMEIVYDEASLEDYINRATELSSDHPVLVDRFLDNAIEIDVDALCDGDEVYLAGVMEHIEEAGIHSGDSACALPPMTLGAQDIEKVREATKKLALGIGVQGLMNVQYALKDDILYVIEANPRASRTVPFVSKATGVNLAKAASRIAVGATIKDLQDEGMIPTEYDGGSLPLDAPIAVKVAVLPFNRFRRPDGKTLDTLLSPEMKSTGEVMGLANNFGAAYAKAEAGAFGALPTEGTVFVTVANRDKRTLILPIQRLASMGYKILATEGTAGMLRRNGIDCEVVLKASDIREGVEGKSIVDRIREGEVDLILNTPAGSAGARHDGYDIRAAAVTVGVPLITTVQGVTAAVQGIEALREGVVSVRALQELDHAVKA

SEQ ID NO: 18 - DNA, 3342 bp, synthetic construct
  misc_feature 1..3342: note = CarB(E918V) NT
  source 1..3342: mol_type = other DNA
atgccaaagcgttcagatattaaccacgtcctcgtcatcggttccggccccatcgtcattggccaggcatgtgaattcgactactccggcacccaggcttgccgcgtgctgaaggaagagggactgcgcgtcaccctcatcaactccaacccagcaacgatcatgaccgacccagaaatggctgaccacacctacgtggagccaatcgagccggaatacatcgacaagattttcgctaaggagatcgagcagggccacccaatcgacgccgtcctggcaacccttggtggccagactgcacttaacgcagctatccagctggatcgcctcggcatcctggaaaagtacggcgttgaactcatcggtgcagacatcgatgccattgagcgcggcgaagatcgccagaagttcaaggatattgtcaccaccatcggtggcgaatccgcgcgttcccgcgtctgccacaacatggacgaagtccatgagactgtcgcagaacttggccttccagtagtcgtgcgtccatccttcactatgggtggcctgggctccggtcttgcatacaacaccgaagaccttgagcgcatcgcaggtggcggacttgctgcatctcctgaagcaaacgtcttgatcgaagaatccatccttggttggaaggaattcgagctcgagctcatgcgcgataccgcagacaacgttgtggttatctgctccattgaaaacgtcgacgcactgggcgtgcacaccggcgactctgtcaccgtggcacctgccctgaccctgactgaccgtgaattccagaagatgcgcgatcagggtatcgccatcatccgcgaggtcggcgtggacaccggtggatgtaacatccagttcgctatcaacccagttgatggccgcatcatcaccattgagatgaacccacgtgtgtctcgttcctccgcgctggcatccaaggcaacgggcttcccaattgccaagatggctgccaagctggctatcggatacaccctggatgagatcaccaacgacatcactggtgaaaccccagctgcgtttgagcccaccatcgactacgtcgtggtcaaggccccacgctttgctttcgagaagtttgtcggcgctgatgacactttgaccaccaccatgaagtccgtcggtgaggtcatgtccctgggccgtaactacattgcagcactgaacaaggcactgcgttccctggaaaccaagcagcagggtttctggaccaagcctgatgagttcttcgcaggggagcgcgctaccgataaggcagctgttctggaagatctcaagcgcccaaccgaaggccgcctctacgacgttgagctggcaatgcgccttggcgcaagcgtggaagaactctacgaagcatcttctattgatccttggttcctcgccgagcttgaagctctcgtgcagttccgccagaagctcgttgacgcaccattcctcaacgaagatctcctgcgcgaagcaaagttcatgggtctgtccgacctgcagatcgcagcccttcgcccagagttcgctggcgaagacggcgtacgcaccttgcgtctgtccctaggcatccgcccagtattcaagactgtggatacctgtgcagcagagtttgaagctaagactccgtaccactactccgcatacgagctggatccagcagctgagtctgaggtcgcaccacagactgagcgtgaaaaggtcctgatcttgggctccggtccaaaccgcatcggccagggcatcgagttcgactattcctgtgttcacgcagctcttgagctctcccgcgtcggctacgaaactgtcatggtcaactgcaacccagagaccgtgtccaccgactacgacaccgctgaccgcctgtacttcgagccactgaccttcgaagacgtcatggaggtctaccacgctgaggcgcagtccggcaccgtcgcaggtgttatcgtccagcttggtggccagactcctctgggcttggcagatcgtttgaagaaggctggcgtccctgtcattggtacctccccagaggcaatcgacatggctgaggaccgtggcgagttcggtgcactgctgaaccgcgagcagcttcctgctccagcattcggcaccgcaacctctttcgaagaggctcgcacagtagccgatgagatcagctacccagtgctggttcgcccttcctacgtcttgggtggccgtggcatggagattgtctacgatgaggcttccctcgaggattacatcaaccgcgcaactgagttgtcttctgaccacccagtgctggttgaccgcttcctggacaacgctattgagatcgacgtcgacgcactgtgcgacggcgacgaagtctacctggcgggcgtcatggaacacatcgaggaagccggcattcactccggtgactccgcatgtgcacttcctccaatgactttgggcgcacaggacatcgagaaggtccgcgaagcaaccaagaagctggctctgggcatcggcgtacagggcctgatgaacgtccagtacgcactcaaggacgacatcctctacgtcatcgaggcaaacccacgtgcatcccgcaccgtgccgttcgtctccaaggcaacgggcgtcaacctggccaaggcagcatcccgtatcgcagtgggcgccaccatcaaggatctccaagatgagggcatgattcctaccgagtacgacggcggctccttgccactggacgctccaatcgctgtgaaggtcgcagtgttgccgttcaaccgcttccgtcgcccagatggaaagaccctggacaccctgctttccccagagatgaagtccactggcgaggtcatgggcttggccaacaacttcggcgctgcatatgcaaaggctgaagctggcgcgtttggtgcattgccaaccgaaggcaccgtcttcgtgaccgtggctaaccgcgacaagcgcaccctgatcctgccaatccagcgcctggcgtcgatgggctacaagatcctcgccaccgaaggcaccgcaggcatgctgcgccgcaacggcattgattgtgaagttgtgctcaaggcttccgacatccgcgaaggtgtagagggcaagtccatcgtggatcgtatccgcgaaggcgaagttgacctcatcctcaacaccccagctggttctgctggcgctcgccacgatggctacgatatccgcgcagcagcagtgaccgtgggtgttccactgatcaccactgtccagggtgtcaccgcagctgtccagggcattgaggccctgcgtgagggcgttgtcagcgtccgcgcgctgcaggaactcgaccacgcagtcaaggcttaa

SEQ ID NO: 19 - protein, 1113 aa, synthetic construct
  REGION 1..1113: note = CarB(T1079A) AA
MPKRSDINHVLVIGSGPIVIGQACEFDYSGTQACRVLKEEGLRVTLINSNPATIMTDPEMADHTYVEPIEPEYIDKIFAKEIEQGHPIDAVLATLGGQTALNAAIQLDRLGILEKYGVELIGADIDAIERGEDRQKFKDIVTTIGGESARSRVCHNMDEVHETVAELGLPVVVRPSFTMGGLGSGLAYNTEDLERIAGGGLAASPEANVLIEESILGWKEFELELMRDTADNVVVICSIENVDALGVHTGDSVTVAPALTLTDREFQKMRDQGIAIIREVGVDTGGCNIQFAINPVDGRIITIEMNPRVSRSSALASKATGFPIAKMAAKLAIGYTLDEITNDITGETPAAFEPTIDYVVVKAPRFAFEKFVGADDTLTTTMKSVGEVMSLGRNYIAALNKALRSLETKQQGFWTKPDEFFAGERATDKAAVLEDLKRPTEGRLYDVELAMRLGASVEELYEASSIDPWFLAELEALVQFRQKLVDAPFLNEDLLREAKFMGLSDLQIAALRPEFAGEDGVRTLRLSLGIRPVFKTVDTCAAEFEAKTPYHYSAYELDPAAESEVAPQTEREKVLILGSGPNRIGQGIEFDYSCVHAALELSRVGYETVMVNCNPETVSTDYDTADRLYFEPLTFEDVMEVYHAEAQSGTVAGVIVQLGGQTPLGLADRLKKAGVPVIGTSPEAIDMAEDRGEFGALLNREQLPAPAFGTATSFEEARTVADEISYPVLVRPSYVLGGRGMEIVYDEASLEDYINRATELSSDHPVLVDRFLDNAIEIDVDALCDGDEVYLAGVMEHIEEAGIHSGDSACALPPMTLGAQDIEKVREATKKLALGIGVQGLMNVQYALKDDILYVIEANPRASRTVPFVSKATGVNLAKAASRIAVGATIKDLQDEGMIPTEYDGGSLPLDAPIAVKEAVLPFNRFRRPDGKTLDTLLSPEMKSTGEVMGLANNFGAAYAKAEAGAFGALPTEGTVFVTVANRDKRTLILPIQRLASMGYKILATEGTAGMLRRNGIDCEVVLKASDIREGVEGKSIVDRIREGEVDLILNTPAGSAGARHDGYDIRAAAVTVGVPLIATVQGVTAAVQGIEALREGVVSVRALQELDHAVKA

SEQ ID NO: 20 - DNA, 3342 bp, synthetic construct
  misc_feature 1..3342: note = CarB(T1079A) NT
  source 1..3342: mol_type = other DNA
atgccaaagcgttcagatattaaccacgtcctcgtcatcggttccggccccatcgtcattggccaggcatgtgaattcgactactccggcacccaggcttgccgcgtgctgaaggaagagggactgcgcgtcaccctcatcaactccaacccagcaacgatcatgaccgacccagaaatggctgaccacacctacgtggagccaatcgagccggaatacatcgacaagattttcgctaaggagatcgagcagggccacccaatcgacgccgtcctggcaacccttggtggccagactgcacttaacgcagctatccagctggatcgcctcggcatcctggaaaagtacggcgttgaactcatcggtgcagacatcgatgccattgagcgcggcgaagatcgccagaagttcaaggatattgtcaccaccatcggtggcgaatccgcgcgttcccgcgtctgccacaacatggacgaagtccatgagactgtcgcagaacttggccttccagtagtcgtgcgtccatccttcactatgggtggcctgggctccggtcttgcatacaacaccgaagaccttgagcgcatcgcaggtggcggacttgctgcatctcctgaagcaaacgtcttgatcgaagaatccatccttggttggaaggaattcgagctcgagctcatgcgcgataccgcagacaacgttgtggttatctgctccattgaaaacgtcgacgcactgggcgtgcacaccggcgactctgtcaccgtggcacctgccctgaccctgactgaccgtgaattccagaagatgcgcgatcagggtatcgccatcatccgcgaggtcggcgtggacaccggtggatgtaacatccagttcgctatcaacccagttgatggccgcatcatcaccattgagatgaacccacgtgtgtctcgttcctccgcgctggcatccaaggcaacgggcttcccaattgccaagatggctgccaagctggctatcggatacaccctggatgagatcaccaacgacatcactggtgaaaccccagctgcgtttgagcccaccatcgactacgtcgtggtcaaggccccacgctttgctttcgagaagtttgtcggcgctgatgacactttgaccaccaccatgaagtccgtcggtgaggtcatgtccctgggccgtaactacattgcagcactgaacaaggcactgcgttccctggaaaccaagcagcagggtttctggaccaagcctgatgagttcttcgcaggggagcgcgctaccgataaggcagctgttctggaagatctcaagcgcccaaccgaaggccgcctctacgacgttgagctggcaatgcgccttggcgcaagcgtggaagaactctacgaagcatcttctattgatccttggttcctcgccgagcttgaagctctcgtgcagttccgccagaagctcgttgacgcaccattcctcaacgaagatctcctgcgcgaagcaaagttcatgggtctgtccgacctgcagatcgcagcccttcgcccagagttcgctggcgaagacggcgtacgcaccttgcgtctgtccctaggcatccgcccagtattcaagactgtggatacctgtgcagcagagtttgaagctaagactccgtaccactactccgcatacgagctggatccagcagctgagtctgaggtcgcaccacagactgagcgtgaaaaggtcctgatcttgggctccggtccaaaccgcatcggccagggcatcgagttcgactattcctgtgttcacgcagctcttgagctctcccgcgtcggctacgaaactgtcatggtcaactgcaacccagagaccgtgtccaccgactacgacaccgctgaccgcctgtacttcgagccactgaccttcgaagacgtcatggaggtctaccacgctgaggcgcagtccggcaccgtcgcaggtgttatcgtccagcttggtggccagactcctctgggcttggcagatcgtttgaagaaggctggcgtccctgtcattggtacctccccagaggcaatcgacatggctgaggaccgtggcgagttcggtgcactgctgaaccgcgagcagcttcctgctccagcattcggcaccgcaacctctttcgaagaggctcgcacagtagccgatgagatcagctacccagtgctggttcgcccttcctacgtcttgggtggccgtggcatggagattgtctacgatgaggcttccctcgaggattacatcaaccgcgcaactgagttgtcttctgaccacccagtgctggttgaccgcttcctggacaacgctattgagatcgacgtcgacgcactgtgcgacggcgacgaagtctacctggcgggcgtcatggaacacatcgaggaagccggcattcactccggtgactccgcatgtgcacttcctccaatgactttgggcgcacaggacatcgagaaggtccgcgaagcaaccaagaagctggctctgggcatcggcgtacagggcctgatgaacgtccagtacgcactcaaggacgacatcctctacgtcatcgaggcaaacccacgtgcatcccgcaccgtgccgttcgtctccaaggcaacgggcgtcaacctggccaaggcagcatcccgtatcgcagtgggcgccaccatcaaggatctccaagatgagggcatgattcctaccgagtacgacggcggctccttgccactggacgctccaatcgctgtgaaggaagcagtgttgccgttcaaccgcttccgtcgcccagatggaaagaccctggacaccctgctttccccagagatgaagtccactggcgaggtcatgggcttggccaacaacttcggcgctgcatatgcaaaggctgaagctggcgcgtttggtgcattgccaaccgaaggcaccgtcttcgtgaccgtggctaaccgcgacaagcgcaccctgatcctgccaatccagcgcctggcgtcgatgggctacaagatcctcgccaccgaaggcaccgcaggcatgctgcgccgcaacggcattgattgtgaagttgtgctcaaggcttccgacatccgcgaaggtgtagagggcaagtccatcgtggatcgtatccgcgaaggcgaagttgacctcatcctcaacaccccagctggttctgctggcgctcgccacgatggctacgatatccgcgcagcagcagtgaccgtgggtgttccactgatcgcaactgtccagggtgtcaccgcagctgtccagggcattgaggccctgcgtgagggcgttgtcagcgtccgcgcgctgcaggaactcgaccacgcagtcaaggcttaa

SEQ ID NO: 21 - protein, 1113 aa, synthetic construct
  REGION 1..1113: note = CarB(T1079I) AA
MPKRSDINHVLVIGSGPIVIGQACEFDYSGTQACRVLKEEGLRVTLINSNPATIMTDPEMADHTYVEPIEPEYIDKIFAKEIEQGHPIDAVLATLGGQTALNAAIQLDRLGILEKYGVELIGADIDAIERGEDRQKFKDIVTTIGGESARSRVCHNMDEVHETVAELGLPVVVRPSFTMGGLGSGLAYNTEDLERIAGGGLAASPEANVLIEESILGWKEFELELMRDTADNVVVICSIENVDALGVHTGDSVTVAPALTLTDREFQKMRDQGIAIIREVGVDTGGCNIQFAINPVDGRIITIEMNPRVSRSSALASKATGFPIAKMAAKLAIGYTLDEITNDITGETPAAFEPTIDYVVVKAPRFAFEKFVGADDTLTTTMKSVGEVMSLGRNYIAALNKALRSLETKQQGFWTKPDEFFAGERATDKAAVLEDLKRPTEGRLYDVELAMRLGASVEELYEASSIDPWFLAELEALVQFRQKLVDAPFLNEDLLREAKFMGLSDLQIAALRPEFAGEDGVRTLRLSLGIRPVFKTVDTCAAEFEAKTPYHYSAYELDPAAESEVAPQTEREKVLILGSGPNRIGQGIEFDYSCVHAALELSRVGYETVMVNCNPETVSTDYDTADRLYFEPLTFEDVMEVYHAEAQSGTVAGVIVQLGGQTPLGLADRLKKAGVPVIGTSPEAIDMAEDRGEFGALLNREQLPAPAFGTATSFEEARTVADEISYPVLVRPSYVLGGRGMEIVYDEASLEDYINRATELSSDHPVLVDRFLDNAIEIDVDALCDGDEVYLAGVMEHIEEAGIHSGDSACALPPMTLGAQDIEKVREATKKLALGIGVQGLMNVQYALKDDILYVIEANPRASRTVPFVSKATGVNLAKAASRIAVGATIKDLQDEGMIPTEYDGGSLPLDAPIAVKEAVLPFNRFRRPDGKTLDTLLSPEMKSTGEVMGLANNFGAAYAKAEAGAFGALPTEGTVFVTVANRDKRTLILPIQRLASMGYKILATEGTAGMLRRNGIDCEVVLKASDIREGVEGKSIVDRIREGEVDLILNTPAGSAGARHDGYDIRAAAVTVGVPLIITVQGVTAAVQGIEALREGVVSVRALQELDHAVKA

SEQ ID NO: 22 - DNA, 3342 bp, synthetic construct
  misc_feature 1..3342: note = CarB(T1079I) NT
  source 1..3342: mol_type = other DNA
atgccaaagcgttcagatattaaccacgtcctcgtcatcggttccggccccatcgtcattggccaggcatgtgaattcgactactccggcacccaggcttgccgcgtgctgaaggaagagggactgcgcgtcaccctcatcaactccaacccagcaacgatcatgaccgacccagaaatggctgaccacacctacgtggagccaatcgagccggaatacatcgacaagattttcgctaaggagatcgagcagggccacccaatcgacgccgtcctggcaacccttggtggccagactgcacttaacgcagctatccagctggatcgcctcggcatcctggaaaagtacggcgttgaactcatcggtgcagacatcgatgccattgagcgcggcgaagatcgccagaagttcaaggatattgtcaccaccatcggtggcgaatccgcgcgttcccgcgtctgccacaacatggacgaagtccatgagactgtcgcagaacttggccttccagtagtcgtgcgtccatccttcactatgggtggcctgggctccggtcttgcatacaacaccgaagaccttgagcgcatcgcaggtggcggacttgctgcatctcctgaagcaaacgtcttgatcgaagaatccatccttggttggaaggaattcgagctcgagctcatgcgcgataccgcagacaacgttgtggttatctgctccattgaaaacgtcgacgcactgggcgtgcacaccggcgactctgtcaccgtggcacctgccctgaccctgactgaccgtgaattccagaagatgcgcgatcagggtatcgccatcatccgcgaggtcggcgtggacaccggtggatgtaacatccagttcgctatcaacccagttgatggccgcatcatcaccattgagatgaacccacgtgtgtctcgttcctccgcgctggcatccaaggcaacgggcttcccaattgccaagatggctgccaagctggctatcggatacaccctggatgagatcaccaacgacatcactggtgaaaccccagctgcgtttgagcccaccatcgactacgtcgtggtcaaggccccacgctttgctttcgagaagtttgtcggcgctgatgacactttgaccaccaccatgaagtccgtcggtgaggtcatgtccctgggccgtaactacattgcagcactgaacaaggcactgcgttccctggaaaccaagcagcagggtttctggaccaagcctgatgagttcttcgcaggggagcgcgctaccgataaggcagctgttctggaagatctcaagcgcccaaccgaaggccgcctctacgacgttgagctggcaatgcgccttggcgcaagcgtggaagaactctacgaagcatcttctattgatccttggttcctcgccgagcttgaagctctcgtgcagttccgccagaagctcgttgacgcaccattcctcaacgaagatctcctgcgcgaagcaaagttcatgggtctgtccgacctgcagatcgcagcccttcgcccagagttcgctggcgaagacggcgtacgcaccttgcgtctgtccctaggcatccgcccagtattcaagactgtggatacctgtgcagcagagtttgaagctaagactccgtaccactactccgcatacgagctggatccagcagctgagtctgaggtcgcaccacagactgagcgtgaaaaggtcctgatcttgggctccggtccaaaccgcatcggccagggcatcgagttcgactattcctgtgttcacgcagctcttgagctctcccgcgtcggctacgaaactgtcatggtcaactgcaacccagagaccgtgtccaccgactacgacaccgctgaccgcctgtacttcgagccactgaccttcgaagacgtcatggaggtctaccacgctgaggcgcagtccggcaccgtcgcaggtgttatcgtccagcttggtggccagactcctctgggcttggcagatcgtttgaagaaggctggcgtccctgtcattggtacctccccagaggcaatcgacatggctgaggaccgtggcgagttcggtgcactgctgaaccgcgagcagcttcctgctccagcattcggcaccgcaacctctttcgaagaggctcgcacagtagccgatgagatcagctacccagtgctggttcgcccttcctacgtcttgggtggccgtggcatggagattgtctacgatgaggcttccctcgaggattacatcaaccgcgcaactgagttgtcttctgaccacccagtgctggttgaccgcttcctggacaacgctattgagatcgacgtcgacgcactgtgcgacggcgacgaagtctacctggcgggcgtcatggaacacatcgaggaagccggcattcactccggtgactccgcatgtgcacttcctccaatgactttgggcgcacaggacatcgagaaggtccgcgaagcaaccaagaagctggctctgggcatcggcgtacagggcctgatgaacgtccagtacgcactcaaggacgacatcctctacgtcatcgaggcaaacccacgtgcatcccgcaccgtgccgttcgtctccaaggcaacgggcgtcaacctggccaaggcagcatcccgtatcgcagtgggcgccaccatcaaggatctccaagatgagggcatgattcctaccgagtacgacggcggctccttgccactggacgctccaatcgctgtgaaggaagcagtgttgccgttcaaccgcttccgtcgcccagatggaaagaccctggacaccctgctttccccagagatgaagtccactggcgaggtcatgggcttggccaacaacttcggcgctgcatatgcaaaggctgaagctggcgcgtttggtgcattgccaaccgaaggcaccgtcttcgtgaccgtggctaaccgcgacaagcgcaccctgatcctgccaatccagcgcctggcgtcgatgggctacaagatcctcgccaccgaaggcaccgcaggcatgctgcgccgcaacggcattgattgtgaagttgtgctcaaggcttccgacatccgcgaaggtgtagagggcaagtccatcgtggatcgtatccgcgaaggcgaagttgacctcatcctcaacaccccagctggttctgctggcgctcgccacgatggctacgatatccgcgcagcagcagtgaccgtgggtgttccactgatcatcactgtccagggtgtcaccgcagctgtccagggcattgaggccctgcgtgagggcgttgtcagcgtccgcgcgctgcaggaactcgaccacgcagtcaaggcttaa

SEQ ID NO: 23 - protein, 1113 aa, synthetic construct
  REGION 1..1113: note = CarB(T1079L) AA
MPKRSDINHVLVIGSGPIVIGQACEFDYSGTQACRVLKEEGLRVTLINSNPATIMTDPEMADHTYVEPIEPEYIDKIFAKEIEQGHPIDAVLATLGGQTALNAAIQLDRLGILEKYGVELIGADIDAIERGEDRQKFKDIVTTIGGESARSRVCHNMDEVHETVAELGLPVVVRPSFTMGGLGSGLAYNTEDLERIAGGGLAASPEANVLIEESILGWKEFELELMRDTADNVVVICSIENVDALGVHTGDSVTVAPALTLTDREFQKMRDQGIAIIREVGVDTGGCNIQFAINPVDGRIITIEMNPRVSRSSALASKATGFPIAKMAAKLAIGYTLDEITNDITGETPAAFEPTIDYVVVKAPRFAFEKFVGADDTLTTTMKSVGEVMSLGRNYIAALNKALRSLETKQQGFWTKPDEFFAGERATDKAAVLEDLKRPTEGRLYDVELAMRLGASVEELYEASSIDPWFLAELEALVQFRQKLVDAPFLNEDLLREAKFMGLSDLQIAALRPEFAGEDGVRTLRLSLGIRPVFKTVDTCAAEFEAKTPYHYSAYELDPAAESEVAPQTEREKVLILGSGPNRIGQGIEFDYSCVHAALELSRVGYETVMVNCNPETVSTDYDTADRLYFEPLTFEDVMEVYHAEAQSGTVAGVIVQLGGQTPLGLADRLKKAGVPVIGTSPEAIDMAEDRGEFGALLNREQLPAPAFGTATSFEEARTVADEISYPVLVRPSYVLGGRGMEIVYDEASLEDYINRATELSSDHPVLVDRFLDNAIEIDVDALCDGDEVYLAGVMEHIEEAGIHSGDSACALPPMTLGAQDIEKVREATKKLALGIGVQGLMNVQYALKDDILYVIEANPRASRTVPFVSKATGVNLAKAASRIAVGATIKDLQDEGMIPTEYDGGSLPLDAPIAVKEAVLPFNRFRRPDGKTLDTLLSPEMKSTGEVMGLANNFGAAYAKAEAGAFGALPTEGTVFVTVANRDKRTLILPIQRLASMGYKILATEGTAGMLRRNGIDCEVVLKASDIREGVEGKSIVDRIREGEVDLILNTPAGSAGARHDGYDIRAAAVTVGVPLILTVQGVTAAVQGIEALREGVVSVRALQELDHAVKA

SEQ ID NO: 24 - DNA, 3342 bp, synthetic construct
  misc_feature 1..3342: note = CarB(T1079L) NT
  source 1..3342: mol_type = other DNA
atgccaaagcgttcagatattaaccacgtcctcgtcatcggttccggccccatcgtcattggccaggcatgtgaattcgactactccggcacccaggcttgccgcgtgctgaaggaagagggactgcgcgtcaccctcatcaactccaacccagcaacgatcatgaccgacccagaaatggctgaccacacctacgtggagccaatcgagccggaatacatcgacaagattttcgctaaggagatcgagcagggccacccaatcgacgccgtcctggcaacccttggtggccagactgcacttaacgcagctatccagctggatcgcctcggcatcctggaaaagtacggcgttgaactcatcggtgcagacatcgatgccattgagcgcggcgaagatcgccagaagttcaaggatattgtcaccaccatcggtggcgaatccgcgcgttcccgcgtctgccacaacatggacgaagtccatgagactgtcgcagaacttggccttccagtagtcgtgcgtccatccttcactatgggtggcctgggctccggtcttgcatacaacaccgaagaccttgagcgcatcgcaggtggcggacttgctgcatctcctgaagcaaacgtcttgatcgaagaatccatccttggttggaaggaattcgagctcgagctcatgcgcgataccgcagacaacgttgtggttatctgctccattgaaaacgtcgacgcactgggcgtgcacaccggcgactctgtcaccgtggcacctgccctgaccctgactgaccgtgaattccagaagatgcgcgatcagggtatcgccatcatccgcgaggtcggcgtggacaccggtggatgtaacatccagttcgctatcaacccagttgatggccgcatcatcaccattgagatgaacccacgtgtgtctcgttcctccgcgctggcatccaaggcaacgggcttcccaattgccaagatggctgccaagctggctatcggatacaccctggatgagatcaccaacgacatcactggtgaaaccccagctgcgtttgagcccaccatcgactacgtcgtggtcaaggccccacgctttgctttcgagaagtttgtcggcgctgatgacactttgaccaccaccatgaagtccgtcggtgaggtcatgtccctgggccgtaactacattgcagcactgaacaaggcactgcgttccctggaaaccaagcagcagggtttctggaccaagcctgatgagttcttcgcaggggagcgcgctaccgataaggcagctgttctggaagatctcaagcgcccaaccgaaggccgcctctacgacgttgagctggcaatgcgccttggcgcaagcgtggaagaactctacgaagcatcttctattgatccttggttcctcgccgagcttgaagctctcgtgcagttccgccagaagctcgttgacgcaccattcctcaacgaagatctcctgcgcgaagcaaagttcatgggtctgtccgacctgcagatcgcagcccttcgcccagagttcgctggcgaagacggcgtacgcaccttgcgtctgtccctaggcatccgcccagtattcaagactgtggatacctgtgcagcagagtttgaagctaagactccgtaccactactccgcatacgagctggatccagcagctgagtctgaggtcgcaccacagactgagcgtgaaaaggtcctgatcttgggctccggtccaaaccgcatcggccagggcatcgagttcgactattcctgtgttcacgcagctcttgagctctcccgcgtcggctacgaaactgtcatggtcaactgcaacccagagaccgtgtccaccgactacgacaccgctgaccgcctgtacttcgagccactgaccttcgaagacgtcatggaggtctaccacgctgaggcgcagtccggcaccgtcgcaggtgttatcgtccagcttggtggccagactcctctgggcttggcagatcgtttgaagaaggctggcgtccctgtcattggtacctccccagaggcaatcgacatggctgaggaccgtggcgagttcggtgcactgctgaaccgcgagcagcttcctgctccagcattcggcaccgcaacctctttcgaagaggctcgcacagtagccgatgagatcagctacccagtgctggttcgcccttcctacgtcttgggtggccgtggcatggagattgtctacgatgaggcttccctcgaggattacatcaaccgcgcaactgagttgtcttctgaccacccagtgctggttgaccgcttcctggacaacgctattgagatcgacgtcgacgcactgtgcgacggcgacgaagtctacctggcgggcgtcatggaacacatcgaggaagccggcattcactccggtgactccgcatgtgcacttcctccaatgactttgggcgcacaggacatcgagaaggtccgcgaagcaaccaagaagctggctctgggcatcggcgtacagggcctgatgaacgtccagtacgcactcaaggacgacatcctctacgtcatcgaggcaaacccacgtgcatcccgcaccgtgccgttcgtctccaaggcaacgggcgtcaacctggccaaggcagcatcccgtatcgcagtgggcgccaccatcaaggatctccaagatgagggcatgattcctaccgagtacgacggcggctccttgccactggacgctccaatcgctgtgaaggaagcagtgttgccgttcaaccgcttccgtcgcccagatggaaagaccctggacaccctgctttccccagagatgaagtccactggcgaggtcatgggcttggccaacaacttcggcgctgcatatgcaaaggctgaagctggcgcgtttggtgcattgccaaccgaaggcaccgtcttcgtgaccgtggctaaccgcgacaagcgcaccctgatcctgccaatccagcgcctggcgtcgatgggctacaagatcctcgccaccgaaggcaccgcaggcatgctgcgccgcaacggcattgattgtgaagttgtgctcaaggcttccgacatccgcgaaggtgtagagggcaagtccatcgtggatcgtatccgcgaaggcgaagttgacctcatcctcaacaccccagctggttctgctggcgctcgccacgatggctacgatatccgcgcagcagcagtgaccgtgggtgttccactgatcctcactgtccagggtgtcaccgcagctgtccagggcattgaggccctgcgtgagggcgttgtcagcgtccgcgcgctgcaggaactcgaccacgcagtcaaggcttaa

SEQ ID NO: 25 - protein, 1113 aa, synthetic construct
  REGION 1..1113: note = CarB(T1079V) AA
MPKRSDINHVLVIGSGPIVIGQACEFDYSGTQACRVLKEEGLRVTLINSNPATIMTDPEMADHTYVEPIEPEYIDKIFAKEIEQGHPIDAVLATLGGQTALNAAIQLDRLGILEKYGVELIGADIDAIERGEDRQKFKDIVTTIGGESARSRVCHNMDEVHETVAELGLPVVVRPSFTMGGLGSGLAYNTEDLERIAGGGLAASPEANVLIEESILGWKEFELELMRDTADNVVVICSIENVDALGVHTGDSVTVAPALTLTDREFQKMRDQGIAIIREVGVDTGGCNIQFAINPVDGRIITIEMNPRVSRSSALASKATGFPIAKMAAKLAIGYTLDEITNDITGETPAAFEPTIDYVVVKAPRFAFEKFVGADDTLTTTMKSVGEVMSLGRNYIAALNKALRSLETKQQGFWTKPDEFFAGERATDKAAVLEDLKRPTEGRLYDVELAMRLGASVEELYEASSIDPWFLAELEALVQFRQKLVDAPFLNEDLLREAKFMGLSDLQIAALRPEFAGEDGVRTLRLSLGIRPVFKTVDTCAAEFEAKTPYHYSAYELDPAAESEVAPQTEREKVLILGSGPNRIGQGIEFDYSCVHAALELSRVGYETVMVNCNPETVSTDYDTADRLYFEPLTFEDVMEVYHAEAQSGTVAGVIVQLGGQTPLGLADRLKKAGVPVIGTSPEAIDMAEDRGEFGALLNREQLPAPAFGTATSFEEARTVADEISYPVLVRPSYVLGGRGMEIVYDEASLEDYINRATELSSDHPVLVDRFLDNAIEIDVDALCDGDEVYLAGVMEHIEEAGIHSGDSACALPPMTLGAQDIEKVREATKKLALGIGVQGLMNVQYALKDDILYVIEANPRASRTVPFVSKATGVNLAKAASRIAVGATIKDLQDEGMIPTEYDGGSLPLDAPIAVKEAVLPFNRFRRPDGKTLDTLLSPEMKSTGEVMGLANNFGAAYAKAEAGAFGALPTEGTVFVTVANRDKRTLILPIQRLASMGYKILATEGTAGMLRRNGIDCEVVLKASDIREGVEGKSIVDRIREGEVDLILNTPAGSAGARHDGYDIRAAAVTVGVPLIVTVQGVTAAVQGIEALREGVVSVRALQELDHAVKA

SEQ ID NO: 26 - DNA, 3342 bp, synthetic construct
  misc_feature 1..3342: note = CarB(T1079V) NT
  source 1..3342: mol_type = other DNA
atgccaaagcgttcagatattaaccacgtcctcgtcatcggttccggccccatcgtcattggccaggcatgtgaattcgactactccggcacccaggcttgccgcgtgctgaaggaagagggactgcgcgtcaccctcatcaactccaacccagcaacgatcatgaccgacccagaaatggctgaccacacctacgtggagccaatcgagccggaatacatcgacaagattttcgctaaggagatcgagcagggccacccaatcgacgccgtcctggcaacccttggtggccagactgcacttaacgcagctatccagctggatcgcctcggcatcctggaaaagtacggcgttgaactcatcggtgcagacatcgatgccattgagcgcggcgaagatcgccagaagttcaaggatattgtcaccaccatcggtggcgaatccgcgcgttcccgcgtctgccacaacatggacgaagtccatgagactgtcgcagaacttggccttccagtagtcgtgcgtccatccttcactatgggtggcctgggctccggtcttgcatacaacaccgaagaccttgagcgcatcgcaggtggcggacttgctgcatctcctgaagcaaacgtcttgatcgaagaatccatccttggttggaaggaattcgagctcgagctcatgcgcgataccgcagacaacgttgtggttatctgctccattgaaaacgtcgacgcactgggcgtgcacaccggcgactctgtcaccgtggcacctgccctgaccctgactgaccgtgaattccagaagatgcgcgatcagggtatcgccatcatccgcgaggtcggcgtggacaccggtggatgtaacatccagttcgctatcaacccagttgatggccgcatcatcaccattgagatgaacccacgtgtgtctcgttcctccgcgctggcatccaaggcaacgggcttcccaattgccaagatggctgccaagctggctatcggatacaccctggatgagatcaccaacgacatcactggtgaaaccccagctgcgtttgagcccaccatcgactacgtcgtggtcaaggccccacgctttgctttcgagaagtttgtcggcgctgatgacactttgaccaccaccatgaagtccgtcggtgaggtcatgtccctgggccgtaactacattgcagcactgaacaaggcactgcgttccctggaaaccaagcagcagggtttctggaccaagcctgatgagttcttcgcaggggagcgcgctaccgataaggcagctgttctggaagatctcaagcgcccaaccgaaggccgcctctacgacgttgagctggcaatgcgccttggcgcaagcgtggaagaactctacgaagcatcttctattgatccttggttcctcgccgagcttgaagctctcgtgcagttccgccagaagctcgttgacgcaccattcctcaacgaagatctcctgcgcgaagcaaagttcatgggtctgtccgacctgcagatcgcagcccttcgcccagagttcgctggcgaagacggcgtacgcaccttgcgtctgtccctaggcatccgcccagtattcaagactgtggatacctgtgcagcagagtttgaagctaagactccgtaccactactccgcatacgagctggatccagcagctgagtctgaggtcgcaccacagactgagcgtgaaaaggtcctgatcttgggctccggtccaaaccgcatcggccagggcatcgagttcgactattcctgtgttcacgcagctcttgagctctcccgcgtcggctacgaaactgtcatggtcaactgcaacccagagaccgtgtccaccgactacgacaccgctgaccgcctgtacttcgagccactgaccttcgaagacgtcatggaggtctaccacgctgaggcgcagtccggcaccgtcgcaggtgttatcgtccagcttggtggccagactcctctgggcttggcagatcgtttgaagaaggctggcgtccctgtcattggtacctccccagaggcaatcgacatggctgaggaccgtggcgagttcggtgcactgctgaaccgcgagcagcttcctgctccagcattcggcaccgcaacctctttcgaagaggctcgcacagtagccgatgagatcagctacccagtgctggttcgcccttcctacgtcttgggtggccgtggcatggagattgtctacgatgaggcttccctcgaggattacatcaaccgcgcaactgagttgtcttctgaccacccagtgctggttgaccgcttcctggacaacgctattgagatcgacgtcgacgcactgtgcgacggcgacgaagtctacctggcgggcgtcatggaacacatcgaggaagccggcattcactccggtgactccgcatgtgcacttcctccaatgactttgggcgcacaggacatcgagaaggtccgcgaagcaaccaagaagctggctctgggcatcggcgtacagggcctgatgaacgtccagtacgcactcaaggacgacatcctctacgtcatcgaggcaaacccacgtgcatcccgcaccgtgccgttcgtctccaaggcaacgggcgtcaacctggccaaggcagcatcccgtatcgcagtgggcgccaccatcaaggatctccaagatgagggcatgattcctaccgagtacgacggcggctccttgccactggacgctccaatcgctgtgaaggaagcagtgttgccgttcaaccgcttccgtcgcccagatggaaagaccctggacaccctgctttccccagagatgaagtccactggcgaggtcatgggcttggccaacaacttcggcgctgcatatgcaaaggctgaagctggcgcgtttggtgcattgccaaccgaaggcaccgtcttcgtgaccgtggctaaccgcgacaagcgcaccctgatcctgccaatccagcgcctggcgtcgatgggctacaagatcctcgccaccgaaggcaccgcaggcatgctgcgccgcaacggcattgattgtgaagttgtgctcaaggcttccgacatccgcgaaggtgtagagggcaagtccatcgtggatcgtatccgcgaaggcgaagttgacctcatcctcaacaccccagctggttctgctggcgctcgccacgatggctacgatatccgcgcagcagcagtgaccgtgggtgttccactgatcgtcactgtccagggtgtcaccgcagctgtccagggcattgaggccctgcgtgagggcgttgtcagcgtccgcgcgctgcaggaactcgaccacgcagtcaaggcttaa

SEQ ID NO: 27 - DNA, 35 bp, synthetic construct
  misc_feature 1..35: note = P18
  source 1..35: mol_type = other DNA
cggtacccggggatcctcttgagctctcccgcgtc

SEQ ID NO: 28 - DNA, 19 bp, synthetic construct
  misc_feature 1..19: note = P19
  source 1..19: mol_type = other DNA
gatgtgttccatgacgccc

SEQ ID NO: 29 - DNA, 38 bp, synthetic construct
  misc_feature 1..38: note = P20
  source 1..38: mol_type = other DNA
ggcgtcatggaacacatcgcagaagccggcattcactc

SEQ ID NO: 30 - DNA, 35 bp, synthetic construct
  misc_feature 1..35: note = P21
  source 1..35: mol_type = other DNA
atgcctgcaggtcgaccgcggttagccacggtcac

SEQ ID NO: 31 - DNA, 38 bp, synthetic construct
  misc_feature 1..38: note = P22
  source 1..38: mol_type = other DNA
ggcgtcatggaacacatcatcgaagccggcattcactc

SEQ ID NO: 32 - DNA, 38 bp, synthetic construct
  misc_feature 1..38: note = P23
  source 1..38: mol_type = other DNA
ggcgtcatggaacacatcctcgaagccggcattcactc

SEQ ID NO: 33 - DNA, 38 bp, synthetic construct
  misc_feature 1..38: note = P24
  source 1..38: mol_type = other DNA
ggcgtcatggaacacatcgtcgaagccggcattcactc

SEQ ID NO: 34 - DNA, 35 bp, synthetic construct
  misc_feature 1..35: note = P25
  source 1..35: mol_type = other DNA
cggtacccggggatccggagattgtctacgatgag

SEQ ID NO: 35 - DNA, 19 bp, synthetic construct
  misc_feature 1..19: note = P26
  source 1..19: mol_type = other DNA
cttcacagcgattggagcg

SEQ ID NO: 36 - DNA, 39 bp, synthetic construct
  misc_feature 1..39: note = P27
  source 1..39: mol_type = other DNA
gctccaatcgctgtgaaggcagcagtgttgccgttcaac

SEQ ID NO: 37 - DNA, 36 bp, synthetic construct
  misc_feature 1..36: note = P28
  source 1..36: mol_type = other DNA
atgcctgcaggtcgacctgacaacgccctcacgcag

SEQ ID NO: 38 - DNA, 39 bp, synthetic construct
  misc_feature 1..39: note = P29
  source 1..39: mol_type = other DNA
gctccaatcgctgtgaagatcgcagtgttgccgttcaac

SEQ ID NO: 39 - DNA, 39 bp, synthetic construct
  misc_feature 1..39: note = P30
  source 1..39: mol_type = other DNA
gctccaatcgctgtgaagctcgcagtgttgccgttcaac

SEQ ID NO: 40 - DNA, 39 bp, synthetic construct
  misc_feature 1..39: note = P31
  source 1..39: mol_type = other DNA
gctccaatcgctgtgaaggtcgcagtgttgccgttcaac

SEQ ID NO: 41 - DNA, 35 bp, synthetic construct
  misc_feature 1..35: note = P32
  source 1..35: mol_type = other DNA
cggtacccggggatcccaaggatctccaagatgag

SEQ ID NO: 42 - DNA, 19 bp, synthetic construct
  misc_feature 1..19: note = P33
  source 1..19: mol_type = other DNA
gatcagtggaacacccacg

SEQ ID NO: 43 - DNA, 38 bp, synthetic construct
  misc_feature 1..38: note = P34
  source 1..38: mol_type = other DNA
gtgggtgttccactgatcgcaactgtccagggtgtcac

SEQ ID NO: 44 - DNA, 35 bp, synthetic construct
  misc_feature 1..35: note = P35
  source 1..35: mol_type = other DNA
atgcctgcaggtcgacctcccctgccgtgttgctc

SEQ ID NO: 45 - DNA, 38 bp, synthetic construct
  misc_feature 1..38: note = P36
  source 1..38: mol_type = other DNA
gtgggtgttccactgatcatcactgtccagggtgtcac

SEQ ID NO: 46 - DNA, 38 bp, synthetic construct
  misc_feature 1..38: note = P37
  source 1..38: mol_type = other DNA
gtgggtgttccactgatcctcactgtccagggtgtcac

SEQ ID NO: 47 - DNA, 38 bp, synthetic construct
  misc_feature 1..38: note = P38
  source 1..38: mol_type = other DNA
gtgggtgttccactgatcgtcactgtccagggtgtcac

SEQ ID NO: 48 - protein, 319 aa, unidentified
  REGION 1..319: note = ArgF
MTSQPQVRHFLADDDLTPAEQAEVLTLAAKLKAAPFSERPLEGPKSVAVLFDKTSTRTRFSFDAGIAHLGGHAIVVDSGSSQMGKGETLQDTAAVLSRYVEAIVWRTYAHSNFHAMAETSTVPLVNSLSDDLHPCQILADLQTIVENLSPEEGPAGLKGKKAVYLGDGDNNMANSYMIGFATAGMDISIIAPEGFQPRAEFVERAEKRGQETGAKVVVTDSLDEVAGADVVITDTWVSMGMENDGIDRTTPFVPYQVNDEVMAKANDGAIFLHCLPAYRGKEVAASVIDGPASKVFDEAENRLHAQKALLVWLLAHQPR

SEQ ID NO: 49 - DNA, 35 bp, synthetic construct
  misc_feature 1..35: note = P4
  source 1..35: mol_type = other DNA
cggtacccggggatcctgaccccaggcaagcacgg

SEQ ID NO: 50 - DNA, 27 bp, synthetic construct
  misc_feature 1..27: note = P5
  source 1..27: mol_type = other DNA
gaagcgagtacgagtttaagtcttatc

SEQ ID NO: 51 - DNA, 20 bp, synthetic construct
  misc_feature 1..20: note = P6
  source 1..20: mol_type = other DNA
aaactcgtactcgcttctcc

SEQ ID NO: 52 - DNA, 35 bp, synthetic construct
  misc_feature 1..35: note = P7
  source 1..35: mol_type = other DNA
atgcctgcaggtcgaccggcgccggcaacctcgtc

SEQ ID NO: 53 - protein, 171 aa, unidentified
  REGION 1..171: note = ArgR
MSLGSTPSTPENLNPVTRTARQALILQILDKQKVTSQVQLSELLLDEGIDITQATLSRDLDELGARKVRPDGGRAYYAVGPVDSIAREDLRGPSEKLRRMLDELLVSTDHSGNIAMLRTPPGAAQYLASFIDRVGLKEVVGTIAGDDTVFVLARDPLTGKELGELLSGRTT

SEQ ID NO: 54 - DNA, 36 bp, synthetic construct
  misc_feature 1..36: note = P8
  source 1..36: mol_type = other DNA
cggtacccggggatccctcgtgcggaattcgtggag

SEQ ID NO: 55 - DNA, 20 bp, synthetic construct
  misc_feature 1..20: note = P9
  source 1..20: mol_type = other DNA
atccagcagcaattcagaca

SEQ ID NO: 56 - DNA, 37 bp, synthetic construct
  misc_feature 1..37: note = P10
  source 1..37: mol_type = other DNA
ctgaattgctgctggattaaggcatcgatatcaccca

SEQ ID NO: 57 - DNA, 36 bp, synthetic construct
  misc_feature 1..36: note = P11
  source 1..36: mol_type = other DNA
atgcctgcaggtcgacccttcattttaagttccttg